European Patent Application EP 4 610 275 A2, published September 3, 2025. Title: ANTI-PD-1 ANTIBODIES AND FUSION PROTEINS. Applicant: Kadmon Corporation, LLC. The sequence listing filed with the application follows.

SEQUENCE LISTING (244 sequences)

SEQ ID NO: 1 - protein, 10 aa, synthetic construct
  REGION 1..10: note = 19B6 HCDR1
GYTFTGYYMH

SEQ ID NO: 2 - protein, 17 aa, synthetic construct
  REGION 1..17: note = 19B6 HCDR2
IINPSGGSTSYAQKFQG

SEQ ID NO: 3 - protein, 15 aa, synthetic construct
  REGION 1..15: note = 19B6 HCDR3
TAGYDWLPSGLGMDV

SEQ ID NO: 4 - protein, 124 aa, synthetic construct
  REGION 1..124: note = 19B6 VH
QVQLVQSGAEVKKPGASVKVSCKASGYTFTGYYMHWVRQAPGQGLEWMGIINPSGGSTSYAQKFQGRVTMTRDTSTSTVYMELSSLRSEDTAVYYCAKTAGYDWLPSGLGMDVWGQGTTVTVSS

SEQ ID NO: 5 - protein, 10 aa, synthetic construct
  REGION 1..10: note = 19B10 HCDR1
GFTFSSYAMH

SEQ ID NO: 6 - protein, 17 aa, synthetic construct
  REGION 1..17: note = 19B10 HCDR2
GISNSGGNTYYADSVKG

SEQ ID NO: 7 - protein, 9 aa, synthetic construct
  REGION 1..9: note = 19B10 HCDR3
DNYYYYMDV

SEQ ID NO: 8 - protein, 118 aa, synthetic construct
  REGION 1..118: note = 19B10 VH
EVQLLESGGGLVQPGGSLRLSCAASGFTFSSYAMHWVRQAPGKGLEWVSGISNSGGNTYYADSVKGRFTISRDNSKNTLYLQMNSLRAEDTAVYYCARDNYYYYMDVWGKGTTVTVSS

SEQ ID NO: 9 - protein, 10 aa, synthetic construct
  REGION 1..10: note = 23A8 HCDR1
GFTFSSSAMH

SEQ ID NO: 10 - protein, 17 aa, synthetic construct
  REGION 1..17: note = 23A8 HCDR2
GISGSGSSTYYADSVKG

SEQ ID NO: 11 - protein, 10 aa, synthetic construct
  REGION 1..10: note = 23A8 HCDR3
DNNYYYYMDV

SEQ ID NO: 12 - protein, 119 aa, synthetic construct
  REGION 1..119: note = 23A8 VH
EVQLLESGGGLVQPGGSLRLSCAASGFTFSSSAMHWVRQAPGKGLEWVSGISGSGSSTYYADSVKGRFTISRDNSKNTLYLQMNSLRAEDTAVYYCARDNNYYYYMDVWGKGTTVTVSS

SEQ ID NO: 13 - protein, 10 aa, synthetic construct
  REGION 1..10: note = 23A11HCDR1
GYTFTDYSLH

SEQ ID NO: 14 - protein, 17 aa, synthetic construct
  REGION 1..17: note = 23A11HCDR2
EVIPMFDTAYYAQTFQG

SEQ ID NO: 15 - protein, 18 aa, synthetic construct
  REGION 1..18: note = 23A11HCDR3
EPFTMVRGGRYYYYGMDV

SEQ ID NO: 16 - protein, 127 aa, synthetic construct
  REGION 1..127: note = 23A11VH
QVQLVQSGAEVKKPGSSVKVSCKASGYTFTDYSLHWVRQAPGQGLEWMGEVIPMFDTAYYAQTFQGRVTITADESTSTAYMELSSLRSEDTAVYYCAREPFTMVRGGRYYYYGMDVWGQGTTVTVSS

SEQ ID NO: 17 - protein, 10 aa, synthetic construct
  REGION 1..10: note = 23H9 HCDR1
GGTFSSSVIS

SEQ ID NO: 18 - protein, 17 aa, synthetic construct
  REGION 1..17: note = 23H9 HCDR2
GIIPIFGTANYAQKFQG

SEQ ID NO: 19 - protein, 20 aa, synthetic construct
  REGION 1..20: note = 23H9 HCDR3
EGLGCSGGSCYSGYYYGMDV

SEQ ID NO: 20 - protein, 129 aa, synthetic construct
  REGION 1..129: note = 23H9 VH
QVQLVQSGAEVKKPGSSVKVSCKASGGTFSSSVISWVRQAPGQGLEWMGGIIPIFGTANYAQKFQGRVTITADESTSTAYMELSSLRSEDTAVYYCAREGLGCSGGSCYSGYYYGMDVWGQGTTVTVSS

SEQ ID NO: 21 - protein, 10 aa, synthetic construct
  REGION 1..10: note = 24H9 HCDR1
GFTFSSYWMS

SEQ ID NO: 22 - protein, 17 aa, synthetic construct
  REGION 1..17: note = 24H9 HCDR2
AISGSGGSTYYADSVKG

SEQ ID NO: 23 - protein, 8 aa, synthetic construct
  REGION 1..8: note = 24H9 HCDR3
SPLQWVDV

SEQ ID NO: 24 - protein, 117 aa, synthetic construct
  REGION 1..117: note = 24H9 VH
EVQLLESGGGLVQPGGSLRLSCAASGFTFSSYWMSWVRQAPGKGLEWVSAISGSGGSTYYADSVKGRFTISRDNSKNTLYLQMNSLRAEDTAVYYCASSPLQWVDVWGQGTTVTVSS

SEQ ID NO: 25 - protein, 11 aa, synthetic construct
  REGION 1..11: note = 19B6 LCDR1
RASQSINSWLA

SEQ ID NO: 26 - protein, 7 aa, synthetic construct
  REGION 1..7: note = 19B6 LCDR2
YASSLQS

SEQ ID NO: 27 - protein, 9 aa, synthetic construct
  REGION 1..9: note = 19B6 LCDR3
QQGYSVPLS

SEQ ID NO: 28 - protein, 107 aa, synthetic construct
  REGION 1..107: note = 19B6 VL
DIQMTQSPSSLSASVGDRVTITCRASQSINSWLAWYQQKPGKAPKLLIYYASSLQSGVPSRFSGSGSGTDFTLTISSLQPEDFATYYCQQGYSVPLSFGQGTKLEIK

SEQ ID NO: 29 - protein, 11 aa, synthetic construct
  REGION 1..11: note = 19B10 LCDR1
RASQSVSTWLA

SEQ ID NO: 30 - protein, 7 aa, synthetic construct
  REGION 1..7: note = 19B10 LCDR2
AASNLET

SEQ ID NO: 31 - protein, 9 aa, synthetic construct
  REGION 1..9: note = 19B10 LCDR3
QQTYSTPYT

SEQ ID NO: 32 - protein, 107 aa, synthetic construct
  REGION 1..107: note = 19B10 VL
DIQMTQSPSSLSASVGDRVTITCRASQSVSTWLAWYQQKPGKAPKLLIYAASNLETGVPSRFSGSGSGTDFTLTISSLQPEDFATYYCQQTYSTPYTFGQGTKLEIK

SEQ ID NO: 33 - protein, 11 aa, synthetic construct
  REGION 1..11: note = 23A8 LCDR1
RASQSIGTWLA

SEQ ID NO: 34 - protein, 7 aa, synthetic construct
  REGION 1..7: note = 23A8 LCDR2
AASTLRS

SEQ ID NO: 35 - protein, 9 aa, synthetic construct
  REGION 1..9: note = 23A8 LCDR3
QQSYSTPYT

SEQ ID NO: 36 - protein, 107 aa, synthetic construct
  REGION 1..107: note = 23A8 VL
DIQMTQSPSSLSASVGDRVTITCRASQSIGTWLAWYQQKPGKAPKLLIYAASTLRSGVPSRFSGSGSGTDFTLTISSLQPEDFATYYCQQSYSTPYTFGQGTKLEIK

SEQ ID NO: 37 - protein, 11 aa, synthetic construct
  REGION 1..11: note = 23A11 LCDR1
RASQNINKNLN

SEQ ID NO: 38 - protein, 7 aa, synthetic construct
  REGION 1..7: note = 23A11 LCDR2 / 39H11 LCDR2
DASNLQS

SEQ ID NO: 39 - protein, 5 aa, synthetic construct
  REGION 1..5: note = 23A11 LCDR3
QHSET

SEQ ID NO: 40 - protein, 103 aa, synthetic construct
  REGION 1..103: note = 23A11 VL
DIQMTQSPSSLSASVGDRVTITCRASQNINKNLNWYQQKPGKAPKLLIYDASNLQSGVPSRFSGSGSGTDFTLTISSLQPEDFATYYCQHSETFGQGTKVEIK

SEQ ID NO: 41 - protein, 16 aa, synthetic construct
  REGION 1..16: note = 23H9 LCDR1 / 31B1 LCDR1 / 33C4 LCDR1 / 33G8 LCDR1
RSSQSLLHSNGYNYLD

SEQ ID NO: 42 - protein, 7 aa, synthetic construct
  REGION 1..7: note = 23H9 LCDR2
LSSHRAS

SEQ ID NO: 43 - protein, 9 aa, synthetic construct
  REGION 1..9: note = 23H9 LCDR3
MQGAHWPYT

SEQ ID NO: 44 - protein, 112 aa, synthetic construct
  REGION 1..112: note = 23H9 VL
DIVMTQSPLSLPVTPGEPASISCRSSQSLLHSNGYNYLDWYLQKPGQSPQLLIYLSSHRASGVPDRFSGSGSGTDFTLKISRVEAEDVGVYYCMQGAHWPYTFGQGTKVEIK

SEQ ID NO: 45 - protein, 11 aa, synthetic construct
  REGION 1..11: note = 24H9 LCDR1
RASQGISSWLA

SEQ ID NO: 46 - protein, 7 aa, synthetic construct
  REGION 1..7: note = 24H9 LCDR2
SASSLQS

SEQ ID NO: 47 - protein, 9 aa, synthetic construct
  REGION 1..9: note = 24H9 LCDR3 / 32G6 LCDR3 / 38A4 LCDR3 / 38A6 LCDR3 / 38A8 LCDR3 /38C11 LCDR3 / 38G11 LCDR3 / 38G9 LCDR3 / 39B11 LCDR3 / 39B3 LCDR3/ 39B6 LCDR3 / 39F11 LCDR3 / 39G5 LCDR3 / 39H2 LCDR3
QQANSFPFT

SEQ ID NO: 48 - protein, 107 aa, synthetic construct
  REGION 1..107: note = 24H9 VL
DIQMTQSPSSLSASVGDRVTITCRASQGISSWLAWYQQKPGKAPKLLIYSASSLQSGVPSRFSGSGSGTDFTLTISSLQPEDFATYYCQQANSFPFTFGPGTKVDIK

SEQ ID NO: 49 - protein, 7 aa, synthetic construct
  REGION 1..7: note = 31B1 LCDR2
EASSLHS

SEQ ID NO: 50 - protein, 9 aa, synthetic construct
  REGION 1..9: note = 31B1 LCDR3
MQGTHWPYT

SEQ ID NO: 51 - protein, 112 aa, synthetic construct
  REGION 1..112: note = 31B1 VL
DIVMTQSPLSLPVTPGEPASISCRSSQSLLHSNGYNYLDWYLQKPGQSPQLLIYEASSLHSGVPDRFSGSGSGTDFTLKISRVEAEDVGVYYCMQGTHWPYTFGQGTKVEIK

SEQ ID NO: 52 - protein, 7 aa, synthetic construct
  REGION 1..7: note = 33C4 LCDR2
EASSLHT

SEQ ID NO: 53 - protein, 9 aa, synthetic construct
  REGION 1..9: note = 33C4 LCDR3
MQGSHWPYT

SEQ ID NO: 54 - protein, 112 aa, synthetic construct
  REGION 1..112: note = 33C4 VL
DIVMTQSPLSLPVTPGEPASISCRSSQSLLHSNGYNYLDWYLQKPGQSPQLLIYEASSLHTGVPDRFSGSGSGTDFTLKISRVEAEDVGVYYCMQGSHWPYTFGQGTKLEIK

SEQ ID NO: 55 - protein, 7 aa, synthetic construct
  REGION 1..7: note = 33G8 LCDR2
QASTLGS

SEQ ID NO: 56 - protein, 9 aa, synthetic construct
  REGION 1..9: note = 33G8 LCDR3
MQGTHWPYT

SEQ ID NO: 57 - protein, 112 aa, synthetic construct
  REGION 1..112: note = 33G8 VL
DIVMTQSPLSLPVTPGEPASISCRSSQSLLHSNGYNYLDWYLQKPGQSPQLLIYQASTLGSGVPDRFSGSGSGTDFTLKISRVEAEDVGVYYCMQGTHWPYTFGQGTKLEIK

SEQ ID NO: 58 - protein, 16 aa, synthetic construct
  REGION 1..16: note = 34C1 LCDR1
RSSESLLYSNGNTYLD

SEQ ID NO: 59 - protein, 7 aa, synthetic construct
  REGION 1..7: note = 34C1 LCDR2
EVSNRAS

SEQ ID NO: 60 - protein, 9 aa, synthetic construct
  REGION 1..9: note = 34C1 LCDR3
MQGTRWPYT

SEQ ID NO: 61 - protein, 112 aa, synthetic construct
  REGION 1..112: note = 34C1 VL
DIVMTQSPLSLPVTPGEPASISCRSSESLLYSNGNTYLDWYLQKPGQSPQLLIYEVSNRASGVPDRFSGSGSGTDFTLKISRVEAEDVGVYYCMQGTRWPYTFGQGTKVEIK

SEQ ID NO: 62 - protein, 16 aa, synthetic construct
  REGION 1..16: note = 23H9 derivatives motif LCDR1
  SITE 4: note = misc_feature - Xaa can be any naturally occurring amino acid
  SITE 8: note = misc_feature - Xaa can be any naturally occurring amino acid
  REGION 12..13: note = misc_feature - Xaa can be any naturally occurring amino acid
RSSXSLLXSNGXXYLD

SEQ ID NO: 63 - skipped

SEQ ID NO: 64 - protein, 9 aa, synthetic construct
  REGION 1..9: note = 23H9 derivatives motif LCDR3
  REGION 4..5: note = misc_feature - Xaa can be any naturally occurring amino acid
MQGXXWPYT

SEQ ID NO: 65 - protein, 112 aa, synthetic construct
  REGION 1..112: note = 23H9 derivatives motif VL
  SITE 27: note = misc_feature - Xaa can be any naturally occurring amino acid
  SITE 31: note = misc_feature - Xaa can be any naturally occurring amino acid
  REGION 35..36: note = misc_feature - Xaa can be any naturally occurring amino acid
  REGION 55..56: note = misc_feature - Xaa can be any naturally occurring amino acid
  REGION 58..61: note = misc_feature - Xaa can be any naturally occurring amino acid
  REGION 97..98: note = misc_feature - Xaa can be any naturally occurring amino acid
DIVMTQSPLSLPVTPGEPASISCRSSXSLLXSNGXXYLDWYLQKPGQSPQLLIYXXSXXXXGVPDRFSGSGSGTDFTLKISRVEAEDVGVYYCMQGXXWPYTFGQGTKVEIK

SEQ ID NO: 66 - protein, 11 aa, synthetic construct
  REGION 1..11: note = 32A11 LCDR1 / 38A8 LCDR1
RASESISIWLA

SEQ ID NO: 67 - protein, 7 aa, synthetic construct
  REGION 1..7: note = 32A11 LCDR2 / 32D11 LCDR2 / 38A8 LCDR2 / 39B3 LCDR2
DASNLET

SEQ ID NO: 68 - protein, 9 aa, synthetic construct
  REGION 1..9: note = 32A11 LCDR3 / 39H11 LCDR3
QQADSFPFT

SEQ ID NO: 69 - protein, 107 aa, synthetic construct
  REGION 1..107: note = 32A11 VL
DIQMTQSPSSLSASVGDRVTITCRASESISIWLAWYQQKPGKAPKLLIYDASNLETGVPSRFSGSGSGTNFTLTISSLQPEDFATYYCQQADSFPFTFGPGTKVDIK

SEQ ID NO: 70 - protein, 11 aa, synthetic construct
  REGION 1..11: note = 32D11 LCDR1
RASQSINIWLA

SEQ ID NO: 71 - protein, 9 aa, synthetic construct
  REGION 1..9: note = 32D11 LCDR3 / 38B10 LCDR3
QQGYSFPFT

SEQ ID NO: 72 - protein, 107 aa, synthetic construct
  REGION 1..107: note = 32D11 VL
DIQMTQSPSSLSASVGDRVTITCRASQSINIWLAWYQQKPGKAPKLLIYDASNLETGVPSRFSGSGSGTDFTLTISSLQPEDFATYYCQQGYSFPFTFGPGTKVDIK

SEQ ID NO: 73 - protein, 11 aa, synthetic construct
  REGION 1..11: note = 32D2 LCDR1
RASQGISRWLA

SEQ ID NO: 74 - protein, 7 aa, synthetic construct
  REGION 1..7: note = 32D2 LCDR2
EASTLQS

SEQ ID NO: 75 - protein, 9 aa, synthetic construct
  REGION 1..9: note = 32D2 LCDR3 / 38B1 LCDR3 / 38H3 LCDR3 / 39G8 LCDR3 / 39H7 LCDR3
QQAYSFPFT

SEQ ID NO: 76 - protein, 107 aa, synthetic construct
  REGION 1..107: note = 32D2 VL
DIQMTQSPSSLSASVGDRVTITCRASQGISRWLAWYQQKPGKAPKLLIYEASTLQSGVPSRFSGSGSGTDFTLTISSLQPEDFATYYCQQAYSFPFTFGQGTKVDIK

SEQ ID NO: 77 - protein, 11 aa, synthetic construct
  REGION 1..11: note = 32G6 LCDR1 / 38A11 LCDR1 / 38A4 LCDR1 / 39A3 LCDR1 / 39B11 LCDR1
RASQSISSWLA

SEQ ID NO: 78 - protein, 7 aa, synthetic construct
  REGION 1..7: note = 32G6 LCDR2 /38A11 LCDR2 / 39F11 LCDR2
DASTLQS

SEQ ID NO: 79 - protein, 107 aa, synthetic construct
  REGION 1..107: note = 32G6 VL
DIQMTQSPSSLSASVGDRVTITCRASQSISSWLAWYQQKPGKAPKLLIYDASTLQSGVPSRFSGSGSGTDFTLTISSLQPEDFATYYCQQANSFPFTFGPGTKVDIK

SEQ ID NO: 80 - protein, 11 aa, synthetic construct
  REGION 1..11: note = 38A10 LCDR1 / 38B1 LCDR1 / 38B10 LCDR1 /39F11 LCDR1
RASQSISTWLA

SEQ ID NO: 81 - protein, 7 aa, synthetic construct
  REGION 1..7: note = 38A10 LCDR2
DASRLQN

SEQ ID NO: 82 - protein, 9 aa, synthetic construct
  REGION 1..9: note = 38A10 LCDR3 / 38B2 LCDR3
QQGDSFPFT

SEQ ID NO: 83 - protein, 107 aa, synthetic construct
  REGION 1..107: note = 38A10 VL
DIQMTQSPSSLSASVGDRVTITCRASQSISTWLAWYQQKPGKAPKLLIYDASRLQNGVPSRFSGSGSGTDFTLTISSLQPEDFATYYCQQGDSFPFTFGPGTKVDIK

SEQ ID NO: 84 - protein, 9 aa, synthetic construct
  REGION 1..9: note = 38A11 LCDR3
QQGNSFPFT

SEQ ID NO: 85 - protein, 107 aa, synthetic construct
  REGION 1..107: note = 38A11 VL
DIQMTQSPSSLSASVGDRVTITCRASQSISSWLAWYQQKPGKAPKLLIYDASTLQSGVPSRFSGSGSGTDFTLTISSLQPEDFATYYCQQGNSFPFTFGPGTKVDIK

SEQ ID NO: 86 - protein, 7 aa, synthetic construct
  REGION 1..7: note = 38A4 LCDR2
DASNLQT

SEQ ID NO: 87 - protein, 107 aa, synthetic construct
  REGION 1..107: note = 38A4 VL
DIQMTQSPSSLSASVGDRVTITCRASQSISSWLAWYQQKPGKAPKLLIYDASNLQTGVPSRFSGSGSGTDFTLTISSLQPEDFATYYCQQANSFPFTFGQGTRLEIK

SEQ ID NO: 88 - protein, 11 aa, synthetic construct
  REGION 1..11: note = 38A6 LCDR1
RASQDISRWLG

SEQ ID NO: 89 - protein, 7 aa, synthetic construct
  REGION 1..7: note = 38A6 LCDR2
AASTLQS

SEQ ID NO: 90 - protein, 107 aa, synthetic construct
  REGION 1..107: note = 38A6 VL
DIQMTQSPSSLSASVGDRVTITCRASQDISRWLGWYQQKPGKAPKLLIYAASTLQSGVPSRFSGSGSGTDFTLTISSLQPEDFATYYCQQANSFPFTFGPGTKLEIK

SEQ ID NO: 91 - protein, 107 aa, synthetic construct
  REGION 1..107: note = 38A8 VL
DIQMTQSPSSLSASVGDRVTITCRASESISIWLAWYQQKPGKAPKLLIYDASNLETGVPSRFSGSGSGTDFTLTISSLQPEDFATYYCQQANSFPFTFGPGTKVDIK

SEQ ID NO: 92 - protein, 7 aa, synthetic construct
  REGION 1..7: note = 38B1 LCDR2
EASKLER

SEQ ID NO: 93 - protein, 107 aa, synthetic construct
  REGION 1..107: note = 38B1 VL
DIQMTQSPSSLSASVGDRVTITCRASQSISTWLAWYQQKPGKAPKLLIYEASKLERGVPSRFSGSGSGTDFTLTISSLQPEDFATYYCQQAYSFPFTFGPGTKVDIK

SEQ ID NO: 94 - protein, 7 aa, synthetic construct
  REGION 1..7: note = 38B10 LCDR2
DASTLQT

SEQ ID NO: 95 - protein, 107 aa, synthetic construct
  REGION 1..107: note = 38B10 VL
DIQMTQSPSSLSASVGDRVTITCRASQSISTWLAWYQQKPGKAPKLLISDASTLQTGVPSRFSGSGSGTDFTLTISSLQPEDFATYYCQQGYSFPFTFGPGTKVDIK

SEQ ID NO: 96 - protein, 11 aa, synthetic construct
  REGION 1..11: note = 38B2 LCDR1
RASESISSWLA

SEQ ID NO: 97 - protein, 7 aa, synthetic construct
  REGION 1..7: note = 38B2 LCDR2
DASSLES

SEQ ID NO: 98 - protein, 107 aa, synthetic construct
  REGION 1..107: note = 38B2 VL
DIQMTQSPSSLSASVGDRVTITCRASESISSWLAWYQQKPGKAPKLLIYDASSLESGVPSRFSGSGSGTDFTLTISSLQPEDFATYYCQQGDSFPFTFGQGTKLEIK

SEQ ID NO: 99 - protein, 11 aa, synthetic construct
  REGION 1..11: note = 38C11 LCDR1
RASQSISRWLA

SEQ ID NO: 100 - protein, 7 aa, synthetic construct
  REGION 1..7: note = 38C11 LCDR2
DASTVQS

SEQ ID NO: 101 - protein, 107 aa, synthetic construct
  REGION 1..107: note = 38C11 VL
DIQMTQSPSSLSASVGDRVTITCRASQSISRWLAWYQQKPGKAPKLLISDASTVQSGVPSRFSGSGSGTDFTLTISSLQPEDFATYYCQQANSFPFTFGPGTKVDIK

SEQ ID NO: 102 - protein, 11 aa, synthetic construct
  REGION 1..11: note = 38C6 LCDR1
RAGRDINKWVA

SEQ ID NO: 103 - protein, 7 aa, synthetic construct
  REGION 1..7: note = 38C6 LCDR2 / 38G11 LCDR2 / 38G9 LCDR2 / 39A3 LCDR2 / 39G5 LCDR2
DASSLQS

SEQ ID NO: 104 - protein, 9 aa, synthetic construct
  REGION 1..9: note = 38C6 LCDR3
QQANSFPFA

SEQ ID NO: 105 - protein, 107 aa, synthetic construct
  REGION 1..107: note = 38C6 VL
DIQMTQSPSSLSASVGDRVTITCRAGRDINKWVAWYQQKPGKAPKLLIYDASSLQSGVPSRFSGSGSGTDFTLTISSLQPEDFATYYCQQANSFPFAFGQGTKVEIK

SEQ ID NO: 106 - protein, 11 aa, synthetic construct
  REGION 1..11: note = 38G11 LCDR1
RASENISRWLA

SEQ ID NO: 107 - protein, 107 aa, synthetic construct
  REGION 1..107: note = 38G11 VL
DIQMTQSPSSLSASVGDRVTITCRASENISRWLAWYQQKPGKAPKLLIYDASSLQSGVPSRFSGSGSGTDFTLTISSLQPEDFATYYCQQANSFPFTFGPGTKVDIK

SEQ ID NO: 108 - protein, 11 aa, synthetic construct
  REGION 1..11: note = 38G9 LCDR1
RVSQSISNWLA

SEQ ID NO: 109 - protein, 97 aa, synthetic construct
  REGION 1..97: note = 38G9 VL
DIQMTQSPSSLSASVGDRVTITCRVSQSISNWLAWYQQKPGKAPKLLIYDASSLQSGVPSRFSGSGSGTDFTLTISSLQPEDFATYYCQQANSFPFT

SEQ ID NO: 110 - protein, 11 aa, synthetic construct
  REGION 1..11: note = 38H3 LCDR1
RASQGISTWLA

SEQ ID NO: 111 - protein, 7 aa, synthetic construct
  REGION 1..7: note = 38H3 LCDR2 / 39B11 LCDR2
EASRLQS

SEQ ID NO: 112 - protein, 107 aa, synthetic construct
  REGION 1..107: note = 38H3 VL
DIQMTQSPSSLSASVGDRVTITCRASQGISTWLAWYQQKPGKAPKLLIYEASRLQSGVPSRFSGSGSGTDFTLTISSLQPEDFATYYCQQAYSFPFTFGPGTKVDIK

SEQ ID NO: 113 - protein, 9 aa, synthetic construct
  REGION 1..9: note = 39A3 LCDR3
QQGDSFPLT

SEQ ID NO: 114 - protein, 107 aa, synthetic construct
  REGION 1..107: note = 39A3 VL
DIQMTQSPSSLSASVGDRVTITCRASQSISSWLAWYQQKPGKAPKLLIYDASSLQSGVPSRFSGSGSGTDFTLTISSLQPEDFATYYCQQGDSFPLTFGQGTKVEIK

SEQ ID NO: 115 - protein, 107 aa, synthetic construct
  REGION 1..107: note = 39B11 VL
DIQMTQSPSSLSASVGDRVTITCRASQSISSWLAWYQQKPGKAPKLLIYEASRLQSGVPSRFSGSGSGTDFTLTISSLQPEDFATYYCQQANSFPFTFGPGTKVDIK

SEQ ID NO: 116 - protein, 11 aa, synthetic construct
  REGION 1..11: note = 39B3 LCDR1
RASQSIGPWLA

SEQ ID NO: 117 - protein, 107 aa, synthetic construct
  REGION 1..107: note = 39B3 VL
DIQMTQSPSSLSASVGDRVTITCRASQSIGPWLAWYQQKPGKAPKLLIYDASNLETGVPSRFSGSGSGTDFTLTISSLQPEDFATYYCQQANSFPFTFGPGTKVDIK

SEQ ID NO: 118 - protein, 11 aa, synthetic construct
  REGION 1..11: note = 39B6 LCDR1
RASEDISHWLA

SEQ ID NO: 119 - protein, 7 aa, synthetic construct
  REGION 1..7: note = 39B6 LCDR2
DAKDLHP

SEQ ID NO: 120 - protein, 107 aa, synthetic construct
  REGION 1..107: note = 39B6 VL
DIQMTQSPSSLSASVGDRVTITCRASEDISHWLAWYQQKPGKAPKLLIYDAKDLHPGVPSRFSGSGSGTDFTLTISSLQPEDFATYYCQQANSFPFTFGQGTRLEIK

SEQ ID NO: 121 - protein, 107 aa, synthetic construct
  REGION 1..107: note = 39F11 VL
DIQMTQSPSSLSASVGDRVTITCRASQSISTWLAWYQQKPGKAPKLLIYDASTLQSGVPSRFSGSGSGTDFTLTISSLQPEDFATYYCQQANSFPFTFGPGTKVDIK

SEQ ID NO: 122 - protein, 11 aa, synthetic construct
  REGION 1..11: note = 39G5 LCDR1
RASQNINVWLA

SEQ ID NO: 123 - protein, 107 aa, synthetic construct
  REGION 1..107: note = 39G5 VL
DIQMTQSPSSLSASVGDRVTITCRASQNINVWLAWYQQKPGKAPKLLIYDASSLQSGVPSRFSGSGSGTDFTLTISSLQPEDFATYYCQQANSFPFTFGPGTKVDIK

SEQ ID NO: 124 - protein, 11 aa, synthetic construct
  REGION 1..11: note = 39G8 LCDR1
RASQGISPWLA

SEQ ID NO: 125 - protein, 7 aa, synthetic construct
  REGION 1..7: note = 39G8 LCDR2
DASKLET

SEQ ID NO: 126 - protein, 107 aa, synthetic construct
  REGION 1..107: note = 39G8 VL
DIQMTQSPSSLSASVGDRVTITCRASQGISPWLAWYQQKPGKAPKLLIYDASKLETGVPSRFSGSGSGTDFTLTISSLQPEDFATYYCQQAYSFPFTFGGGTKVEIK

SEQ ID NO: 127 - protein, 11 aa, synthetic construct
  REGION 1..11: note = 39H11 LCDR1
RASQSIGIWVA

SEQ ID NO: 128 - protein, 107 aa, synthetic construct
  REGION 1..107: note = 39H11 VL
DIQMTQSPSSLSASVGDRVTITCRASQSIGIWVAWYQQKPGKAPKLLIYDASNLQSGVPSRFSGSGSGTDFTLTISSLQPEDFATYYCQQADSFPFTFGQGTKVEIK

SEQ ID NO: 129 - protein, 11 aa, synthetic construct
  REGION 1..11: note = 39H2 LCDR1
RASQNIGPWLA

SEQ ID NO: 130 - protein, 7 aa, synthetic construct
  REGION 1..7: note = 39H2 LCDR2
DASTLHS

SEQ ID NO: 131 - protein, 107 aa, synthetic construct
  REGION 1..107: note = 39H2 VL
DIQMTQSPSSLSASVGDRVTITCRASQNIGPWLAWYQQKPGKAPKLLIYDASTLHSGVPSRFSGSGSGTDFTLTISSLQPEDFATYYCQQANSFPFTFGQGTRLEIK

SEQ ID NO: 132 - protein, 11 aa, synthetic construct
  REGION 1..11: note = 39H7 LCDR1
RASQSISNWLA

SEQ ID NO: 133 - protein, 7 aa, synthetic construct
  REGION 1..7: note = 39H7 LCDR2
DASNLQA

SEQ ID NO: 134 - protein, 107 aa, synthetic construct
  REGION 1..107: note = 39H7 VL
DIQMTQSPSSLSASVGDRVTITCRASQSISNWLAWYQQKPGKAPKLLIYDASNLQAGVPSRFSGSGSGTDFTLTISSLQPEDFATYYCQQAYSFPFTFGPGTKVDIK

SEQ ID NO: 135 - protein, 11 aa, synthetic construct
  REGION 1..11: note = 24H9 derivatives motif LCR1
  REGION 3..5: note = misc_feature - Xaa can be any naturally occurring amino acid
  REGION 7..8: note = misc_feature - Xaa can be any naturally occurring amino acid
  SITE 10: note = misc_feature - Xaa can be any naturally occurring amino acid
RAXXXIXXWXA

SEQ ID NO: 136 - skipped

SEQ ID NO: 137 - protein, 9 aa, synthetic construct
  REGION 1..9: note = 24H9 derivatives motif LCR3
  REGION 3..4: note = misc_feature - Xaa can be any naturally occurring amino acid
  REGION 8..9: note = misc_feature - Xaa can be any naturally occurring amino acid
QQXXSFPXX

SEQ ID NO: 138 - protein, 107 aa, synthetic construct
  REGION 1..107: note = 24H9 derivatives motif VL
  REGION 26..28: note = misc_feature - Xaa can be any naturally occurring amino acid
  REGION 30..31: note = misc_feature - Xaa can be any naturally occurring amino acid
  SITE 33: note = misc_feature - Xaa can be any naturally occurring amino acid
  SITE 50: note = misc_feature - Xaa can be any naturally occurring amino acid
  REGION 53..56: note = misc_feature - Xaa can be any naturally occurring amino acid
  REGION 91..92: note = misc_feature - Xaa can be any naturally occurring amino acid
  REGION 96..97: note = misc_feature - Xaa can be any naturally occurring amino acid
DIQMTQSPSSLSASVGDRVTITCRAXXXIXXWXAWYQQKPGKAPKLLIYXASXXXXGVPSRFSGSGSGTDFTLTISSLQPEDFATYYCQQXXSFPXXFGPGTKVDIK

SEQ ID NO: 139 - protein, 10 aa, synthetic construct
  REGION 1..10: note = R3A9 HCDR1
GHTFTSYYIH

SEQ ID NO: 140 - protein, 18 aa, synthetic construct
  REGION 1..18: note = R3A9 HCDR2
GIINPSGGSTSYAQKFQG

SEQ ID NO: 141 - protein, 10 aa, synthetic construct
  REGION 1..10: note = R3A9 HCDR3
DRAYGGAGDY

SEQ ID NO: 142 - protein, 119 aa, synthetic construct
  REGION 1..119: note = R3A9 VH
QVQLVQSGAEVKKPGASVKVSCKASGHTFTSYYIHWVRQAPGQGLEWMGIINPSGGSTSYAQKFQGRVTMTRDTSTSTVYMELSSLRSEDTAVYYCARDRAYGGAGDYWGQGTLVTVSS

SEQ ID NO: 143 - protein, 11 aa, synthetic construct
  REGION 1..11: note = R3A9 LCDR1
RASQSVGTWLA

SEQ ID NO: 144 - protein, 7 aa, synthetic construct
  REGION 1..7: note = R3A9 LCDR2
SASTLQS

SEQ ID NO: 145 - protein, 9 aa, synthetic construct
  REGION 1..9: note = R3A9 LCDR3
QQSYSAPLT

SEQ ID NO: 146 - protein, 107 aa, synthetic construct
  REGION 1..107: note = R3A9 VL
DIQMTQSPSSLSASVGDRVTITCRASQSVGTWLAWYQQKPGKAPKLLIYSASTLQSGVPSRFSGSGSGTDFTLTISSLQPEDFATYYCQQSYSAPLTFGGGTKVEIK

SEQ ID NO: 147 - protein, 11 aa, synthetic construct
  REGION 1..11: note = m3A7 LCDR1
RASRSISNWLA

SEQ ID NO: 148 - protein, 7 aa, synthetic construct
  REGION 1..7: note = m3A7 LCDR2 / m2C1 LCDR2
AASSLQS

SEQ ID NO: 149 - protein, 9 aa, synthetic construct
  REGION 1..9: note = m3A7 LCDR3
QQSYSAPVT

SEQ ID NO: 150 - protein, 107 aa, synthetic construct
  REGION 1..107: note = m3A7 VL
DIQMTQSPSSLSASVGDRVTITCRASRSISNWLAWYQQKPGKAPKLLIYAASSLQSGVPSRFSGSGSGTDFTLTISSLQPEDFATYYCQQSYSAPVTFGQGTKVEIK

SEQ ID NO: 151 - protein, 11 aa, synthetic construct
  REGION 1..11: note = m2C1 LCDR1
RASRSISSWLA

SEQ ID NO: 152 - protein, 9 aa, synthetic construct
  REGION 1..9: note = m2C1 LCDR3
QQSYSIPAT

SEQ ID NO: 153 - protein, 107 aa, synthetic construct
  REGION 1..107: note = m2C1 VL
DIQMTQSPSSLSASVGDRVTITCRASRSISSWLAWYQQKPGKAPKLLIYAASSLQSGVPSRFSGSGSGTDFTLTISSLQPEDFATYYCQQSYSIPATFGQGTKVEIK

SEQ ID NO: 154 - protein, 11 aa, synthetic construct
  REGION 1..11: note = m2A1 LCDR1
RASRGISSWLA

SEQ ID NO: 155 - protein, 9 aa, synthetic construct
  REGION 1..9: note = m2A1 LCDR3
QQSYSPPWT

SEQ ID NO: 156 - protein, 107 aa, synthetic construct
  REGION 1..107: note = m2A1 VL
DIQMTQSPSSLSASVGDRVTITCRASRGISSWLAWYQQKPGKAPKLLIYAASSLQSGVPSRFSGSGSGTDFTLTISSLQPEDFATYYCQQSYSPPWTFGQGTKVEIK

SEQ ID NO: 157 - protein, 11 aa, synthetic construct
  REGION 1..11: note = m4A5 LCDR1 / m3C6 LCDR1
RASQSIDTWLA

SEQ ID NO: 158 - protein, 7 aa, synthetic construct
  REGION 1..7: note = m4A5 LCDR2
AASTLES

SEQ ID NO: 159 - protein, 9 aa, synthetic construct
  REGION 1..9: note = m4A5 LCDR3
QQSYRAPLT

SEQ ID NO: 160 - protein, 107 aa, synthetic construct
  REGION 1..107: note = m4A5 VL
DIQMTQSPSSLSASVGDRVTITCRASQSIDTWLAWYQQKPGKAPKLLIYAASTLESGVPSRFSGSGSGTDFTLTISSLQPEDFATYYCQQSYRAPLTFGQGTKVEIK

SEQ ID NO: 161 - protein, 11 aa, synthetic construct
  REGION 1..11: note = m4D1 LCDR1
RASQSISAWLA

SEQ ID NO: 162 - protein, 7 aa, synthetic construct
  REGION 1..7: note = m4D1 LCDR2
KASSLES

SEQ ID NO: 163 - protein, 9 aa, synthetic construct
  REGION 1..9: note = m4D1 LCDR3
QQSYSPPAT

SEQ ID NO: 164 - protein, 107 aa, synthetic construct
  REGION 1..107: note = m4D1 VL
DIQMTQSPSSLSASVGDRVTITCRASQSISAWLAWYQQKPGKAPKLLIYKASSLESGVPSRFSGSGSGTDFTLTISSLQPEDFATYYCQQSYSPPATFGGGTKVEIK

SEQ ID NO: 165 - protein, 7 aa, synthetic construct
  REGION 1..7: note = m3C6 LCDR2
EASSLQG

SEQ ID NO: 166 - protein, 8 aa, synthetic construct
  REGION 1..8: note = m3C6 LCDR3
QQSYSTWT

SEQ ID NO: 167 - protein, 106 aa, synthetic construct
  REGION 1..106: note = m3C6 VL
DIQMTQSPSSLSASVGDRVTITCRASQSIDTWLAWYQQKPGKAPKLLIYEASSLQGGVPSRFSGSGSGTDFTLTISSLQPEDFATYYCQQSYSTWTFGQGTKVEIK

SEQ ID NO: 168 - protein, 447 aa, synthetic construct
  REGION 1..447: note = 38B2 full length HC
EVQLLESGGGLVQPGGSLRLSCAASGFTFSSYWMSWVRQAPGKGLEWVSAISGSGGSTYYADSVKGRFTISRDNSKNTLYLQMNSLRAEDTAVYYCASSPLQWVDVWGQGTTVTVSSASTKGPSVFPLAPSSKSTSGGTAALGCLVKDYFPEPVTVSWNSGALTSGVHTFPAVLQSSGLYSLSSVVTVPSSSLGTQTYICNVNHKPSNTKVDKRVEPKSCDKTHTCPPCPAPELLGGPSVFLFPPKPKDTLMISRTPEVTCVVVDVSHEDPEVKFNWYVDGVEVHNAKTKPREEQYNSTYRVVSVLTVLHQDWLNGKEYKCKVSNKALPAPIEKTISKAKGQPREPQVYTLPPSREEMTKNQVSLTCLVKGFYPSDIAVEWESNGQPENNYKTTPPVLDSDGSFFLYSKLTVDKSRWQQGNVFSCSVMHEALHNHYTQKSLSLSPGK

SEQ ID NO: 169 - protein, 447 aa, synthetic construct
  REGION 1..447: note = 38B2 HC (T350V/T366L/ K392L/ T394W) LALAPG
EVQLLESGGGLVQPGGSLRLSCAASGFTFSSYWMSWVRQAPGKGLEWVSAISGSGGSTYYADSVKGRFTISRDNSKNTLYLQMNSLRAEDTAVYYCASSPLQWVDVWGQGTTVTVSSASTKGPSVFPLAPSSKSTSGGTAALGCLVKDYFPEPVTVSWNSGALTSGVHTFPAVLQSSGLYSLSSVVTVPSSSLGTQTYICNVNHKPSNTKVDKRVEPKSCDKTHTCPPCPAPEAAGGPSVFLFPPKPKDTLMISRTPEVTCVVVDVSHEDPEVKFNWYVDGVEVHNAKTKPREEQYNSTYRVVSVLTVLHQDWLNGKEYKCKVSNKALGAPIEKTISKAKGQPREPQVYVLPPSREEMTKNQVSLLCLVKGFYPSDIAVEWESNGQPENNYLTWPPVLDSDGSFFLYSKLTVDKSRWQQGNVFSCSVMHEALHNHYTQKSLSLSPGK

SEQ ID NO: 170 - protein, 214 aa, synthetic construct
  REGION 1..214: note = 38B2 full length LC
DIQMTQSPSSLSASVGDRVTITCRASESISSWLAWYQQKPGKAPKLLIYDASSLESGVPSRFSGSGSGTDFTLTISSLQPEDFATYYCQQGDSFPFTFGQGTKLEIKRTVAAPSVFIFPPSDEQLKSGTASVVCLLNNFYPREAKVQWKVDNALQSGNSQESVTEQDSKDSTYSLSSTLTLSKADYEKHKVYACEVTHQGLSSPVTKSFNRGEC

SEQ ID NO: 171 - protein, 449 aa, synthetic construct
  REGION 1..449: note = m3A7 full length mHC LALAPG
QVQLVQSGAEVKKPGASVKVSCKASGHTFTSYYIHWVRQAPGQGLEWMGIINPSGGSTSYAQKFQGRVTMTRDTSTSTVYMELSSLRSEDTAVYYCARDRAYGGAGDYWGQGTLVTVSSAKTTAPSVYPLAPVCGDTTGSSVTLGCLVKGYFPEPVTLTWNSGSLSSGVHTFPAVLQSDLYTLSSSVTVTSSTWPSQSITCNVAHPASSTKVDKKIEPRGPTIKPCPPCKCPAPNAAGGPSVFIFPPKIKDVLMISLSPIVTCVVVDVSEDDPDVQISWFVNNVEVHTAQTQTHREDYNSTLRVVSALPIQHQDWMSGKEFKCKVNNKDLGAPIERTISKPKGSVRAPQVYVLPPPEEEMTKKQVTLTCMVTDFMPEDIYVEWTNNGKTELNYKNTEPVLDSDGSYFMYSKLRVEKKNWVERNSYSCSVVHEGLHNHHTTKSFSRTPGK

SEQ ID NO: 172 - protein, 449 aa, synthetic construct
  REGION 1..449: note = m3A7 mHC (L351Y/F405A/Y407V) LALAPG
QVQLVQSGAEVKKPGASVKVSCKASGHTFTSYYIHWVRQAPGQGLEWMGIINPSGGSTSYAQKFQGRVTMTRDTSTSTVYMELSSLRSEDTAVYYCARDRAYGGAGDYWGQGTLVTVSSAKTTAPSVYPLAPVCGDTTGSSVTLGCLVKGYFPEPVTLTWNSGSLSSGVHTFPAVLQSDLYTLSSSVTVTSSTWPSQSITCNVAHPASSTKVDKKIEPRGPTIKPCPPCKCPAPNAAGGPSVFIFPPKIKDVLMISLSPIVTCVVVDVSEDDPDVQISWFVNNVEVHTAQTQTHREDYNSTLRVVSALPIQHQDWMSGKEFKCKVNNKDLGAPIERTISKPKGSVRAPQVYVYPPPEEEMTKKQVTLTCMVTDFMPEDIYVEWTNNGKTELNYKNTEPVLDSDGSYAMVSKLRVEKKNWVERNSYSCSVVHEGLHNHHTTKSFSRTPGK

SEQ ID NO: 173 - protein, 214 aa, synthetic construct
  REGION 1..214: note = m3A7 full length mLC
DIQMTQSPSSLSASVGDRVTITCRASRSISNWLAWYQQKPGKAPKLLIYAASSLQSGVPSRFSGSGSGTDFTLTISSLQPEDFATYYCQQSYSAPVTFGQGTKVEIKRADAAPTVSIFPPSSEQLTSGGASVVCFLNNFYPKDINVKWKIDGSERQNGVLNSWTDQDSKDSTYSMSSTLTLTKDEYERHNSYTCEATHKTSTSPIVKSFNRNEC

SEQ ID NO: 174 - protein, 688 aa, synthetic construct
  REGION 1..688: note = hSD15 + 38B2 HCLALAPG
ITCPPPMSVEHADIWVKSYSLYSRERYICNSGFKRKAGTSSLTECVLNKATNVAHWTTPSLKCIRDPALVHQRPAPPSGGSGGGGSGGGSGGGGSLQNWVNVISDLKKIEDLIQSMHIDATLYTESDVHPSCKVTAMKCFLLELQVISLESGDASIHDTVENLIILANNSLSSNGNVTESGCKECEELEEKNIKEFLQSFVHIVQMFINTSGGGGSGGGGSGGGGSGGGGSGGGGSGGGGSEVQLLESGGGLVQPGGSLRLSCAASGFTFSSYWMSWVRQAPGKGLEWVSAISGSGGSTYYADSVKGRFTISRDNSKNTLYLQMNSLRAEDTAVYYCASSPLQWVDVWGQGTTVTVSSASTKGPSVFPLAPSSKSTSGGTAALGCLVKDYFPEPVTVSWNSGALTSGVHTFPAVLQSSGLYSLSSVVTVPSSSLGTQTYICNVNHKPSNTKVDKRVEPKSCDKTHTCPPCPAPEAAGGPSVFLFPPKPKDTLMISRTPEVTCVVVDVSHEDPEVKFNWYVDGVEVHNAKTKPREEQYNSTYRVVSVLTVLHQDWLNGKEYKCKVSNKALGAPIEKTISKAKGQPREPQVYTLPPSREEMTKNQVSLTCLVKGFYPSDIAVEWESNGQPENNYKTTPPVLDSDGSFFLYSKLTVDKSRWQQGNVFSCSVMHEALHNHYTQKSLSLSPGK

SEQ ID NO: 175 - protein, 688 aa, synthetic construct
  REGION 1..688: note = hSD15 + 38B2HC (T350V/L351Y/F405A/Y407V) LALAPG
ITCPPPMSVEHADIWVKSYSLYSRERYICNSGFKRKAGTSSLTECVLNKATNVAHWTTPSLKCIRDPALVHQRPAPPSGGSGGGGSGGGSGGGGSLQNWVNVISDLKKIEDLIQSMHIDATLYTESDVHPSCKVTAMKCFLLELQVISLESGDASIHDTVENLIILANNSLSSNGNVTESGCKECEELEEKNIKEFLQSFVHIVQMFINTSGGGGSGGGGSGGGGSGGGGSGGGGSGGGGSEVQLLESGGGLVQPGGSLRLSCAASGFTFSSYWMSWVRQAPGKGLEWVSAISGSGGSTYYADSVKGRFTISRDNSKNTLYLQMNSLRAEDTAVYYCASSPLQWVDVWGQGTTVTVSSASTKGPSVFPLAPSSKSTSGGTAALGCLVKDYFPEPVTVSWNSGALTSGVHTFPAVLQSSGLYSLSSVVTVPSSSLGTQTYICNVNHKPSNTKVDKRVEPKSCDKTHTCPPCPAPEAAGGPSVFLFPPKPKDTLMISRTPEVTCVVVDVSHEDPEVKFNWYVDGVEVHNAKTKPREEQYNSTYRVVSVLTVLHQDWLNGKEYKCKVSNKALGAPIEKTISKAKGQPREPQVYVYPPSREEMTKNQVSLTCLVKGFYPSDIAVEWESNGQPENNYKTTPPVLDSDGSFALVSKLTVDKSRWQQGNVFSCSVMHEALHNHYTQKSLSLSPGK

SEQ ID NO: 176 - protein, 656 aa, synthetic construct
  REGION 1..656: note = 38B2HC LALAPG + hSD15
EVQLLESGGGLVQPGGSLRLSCAASGFTFSSYWMSWVRQAPGKGLEWVSAISGSGGSTYYADSVKGRFTISRDNSKNTLYLQMNSLRAEDTAVYYCASSPLQWVDVWGQGTTVTVSSASTKGPSVFPLAPSSKSTSGGTAALGCLVKDYFPEPVTVSWNSGALTSGVHTFPAVLQSSGLYSLSSVVTVPSSSLGTQTYICNVNHKPSNTKVDKRVEPKSCDKTHTCPPCPAPEAAGGPSVFLFPPKPKDTLMISRTPEVTCVVVDVSHEDPEVKFNWYVDGVEVHNAKTKPREEQYNSTYRVVSVLTVLHQDWLNGKEYKCKVSNKALGAPIEKTISKAKGQPREPQVYTLPPSREEMTKNQVSLTCLVKGFYPSDIAVEWESNGQPENNYKTTPPVLDSDGSFFLYSKLTVDKSRWQQGNVFSCSVMHEALHNHYTQKSLSLSPGSCPPPMSVEHADIWVKSYSLYSRERYICNSGFKRKAGTSSLTECVLNKATNVAHWTTPSLKCIRDPALVHQRPAPPSGGSGGGGSGGGSGGGGSLQNWVNVISDLKKIEDLIQSMHIDATLYTESDVHPSCKVTAMKCFLLELQVISLESGDASIHDTVENLIILANNSLSSNGNVTESGCKECEELEEKNIKEFLQSFVHIVQMFINTS

SEQ ID NO: 177 - protein, 656 aa, synthetic construct
  REGION 1..656: note = 38B2 HC (T350V/L351Y/F405A/Y407V) LALAPG + hSD15
EVQLLESGGGLVQPGGSLRLSCAASGFTFSSYWMSWVRQAPGKGLEWVSAISGSGGSTYYADSVKGRFTISRDNSKNTLYLQMNSLRAEDTAVYYCASSPLQWVDVWGQGTTVTVSSASTKGPSVFPLAPSSKSTSGGTAALGCLVKDYFPEPVTVSWNSGALTSGVHTFPAVLQSSGLYSLSSVVTVPSSSLGTQTYICNVNHKPSNTKVDKRVEPKSCDKTHTCPPCPAPEAAGGPSVFLFPPKPKDTLMISRTPEVTCVVVDVSHEDPEVKFNWYVDGVEVHNAKTKPREEQYNSTYRVVSVLTVLHQDWLNGKEYKCKVSNKALGAPIEKTISKAKGQPREPQVYVYPPSREEMTKNQVSLTCLVKGFYPSDIAVEWESNGQPENNYKTTPPVLDSDGSFALVSKLTVDKSRWQQGNVFSCSVMHEALHNHYTQKSLSLSPGSCPPPMSVEHADIWVKSYSLYSRERYICNSGFKRKAGTSSLTECVLNKATNVAHWTTPSLKCIRDPALVHQRPAPPSGGSGGGGSGGGSGGGGSLQNWVNVISDLKKIEDLIQSMHIDATLYTESDVHPSCKVTAMKCFLLELQVISLESGDASIHDTVENLIILANNSLSSNGNVTESGCKECEELEEKNIKEFLQSFVHIVQMFINTS

SEQ ID NO: 178 - protein, 688 aa, synthetic construct
  REGION 1..688: note = N65A_hSD15+38B2 HC (T350V/L351Y/F405A/Y407V) LALAPG
ITCPPPMSVEHADIWVKSYSLYSRERYICNSGFKRKAGTSSLTECVLNKATNVAHWTTPSLKCIRDPALVHQRPAPPSGGSGGGGSGGGSGGGGSLQNWVNVISDLKKIEDLIQSMHIDATLYTESDVHPSCKVTAMKCFLLELQVISLESGDASIHDTVEALIILANNSLSSNGNVTESGCKECEELEEKNIKEFLQSFVHIVQMFINTSGGGGSGGGGSGGGGSGGGGSGGGGSGGGGSEVQLLESGGGLVQPGGSLRLSCAASGFTFSSYWMSWVRQAPGKGLEWVSAISGSGGSTYYADSVKGRFTISRDNSKNTLYLQMNSLRAEDTAVYYCASSPLQWVDVWGQGTTVTVSSASTKGPSVFPLAPSSKSTSGGTAALGCLVKDYFPEPVTVSWNSGALTSGVHTFPAVLQSSGLYSLSSVVTVPSSSLGTQTYICNVNHKPSNTKVDKRVEPKSCDKTHTCPPCPAPEAAGGPSVFLFPPKPKDTLMISRTPEVTCVVVDVSHEDPEVKFNWYVDGVEVHNAKTKPREEQYNSTYRVVSVLTVLHQDWLNGKEYKCKVSNKALGAPIEKTISKAKGQPREPQVYVYPPSREEMTKNQVSLTCLVKGFYPSDIAVEWESNGQPENNYKTTPPVLDSDGSFALVSKLTVDKSRWQQGNVFSCSVMHEALHNHYTQKSLSLSPGK

SEQ ID NO: 179 - protein, 688 aa, synthetic construct
  REGION 1..688: note = N65D_hSD15 + 38B2 HC (T350V/L351Y/F405A/Y407V) LALAPG
ITCPPPMSVEHADIWVKSYSLYSRERYICNSGFKRKAGTSSLTECVLNKATNVAHWTTPSLKCIRDPALVHQRPAPPSGGSGGGGSGGGSGGGGSLQNWVNVISDLKKIEDLIQSMHIDATLYTESDVHPSCKVTAMKCFLLELQVISLESGDASIHDTVEDLIILANNSLSSNGNVTESGCKECEELEEKNIKEFLQSFVHIVQMFINTSGGGGSGGGGSGGGGSGGGGSGGGGSGGGGSEVQLLESGGGLVQPGGSLRLSCAASGFTFSSYWMSWVRQAPGKGLEWVSAISGSGGSTYYADSVKGRFTISRDNSKNTLYLQMNSLRAEDTAVYYCASSPLQWVDVWGQGTTVTVSSASTKGPSVFPLAPSSKSTSGGTAALGCLVKDYFPEPVTVSWNSGALTSGVHTFPAVLQSSGLYSLSSVVTVPSSSLGTQTYICNVNHKPSNTKVDKRVEPKSCDKTHTCPPCPAPEAAGGPSVFLFPPKPKDTLMISRTPEVTCVVVDVSHEDPEVKFNWYVDGVEVHNAKTKPREEQYNSTYRVVSVLTVLHQDWLNGKEYKCKVSNKALGAPIEKTISKAKGQPREPQVYVYPPSREEMTKNQVSLTCLVKGFYPSDIAVEWESNGQPENNYKTTPPVLDSDGSFALVSKLTVDKSRWQQGNVFSCSVMHEALHNHYTQKSLSLSPGK

SEQ ID NO: 180 - protein, 688 aa, synthetic construct
  REGION 1..688: note = N65S_hSD15+38B2 HC (T350V/L351Y/F405A/Y407V)
ITCPPPMSVEHADIWVKSYSLYSRERYICNSGFKRKAGTSSLTECVLNKATNVAHWTTPSLKCIRDPALVHQRPAPPSGGSGGGGSGGGSGGGGSLQNWVNVISDLKKIEDLIQSMHIDATLYTESDVHPSCKVTAMKCFLLELQVISLESGDASIHDTVESLIILANNSLSSNGNVTESGCKECEELEEKNIKEFLQSFVHIVQMFINTSGGGGSGGGGSGGGGSGGGGSGGGGSGGGGSEVQLLESGGGLVQPGGSLRLSCAASGFTFSSYWMSWVRQAPGKGLEWVSAISGSGGSTYYADSVKGRFTISRDNSKNTLYLQMNSLRAEDTAVYYCASSPLQWVDVWGQGTTVTVSSASTKGPSVFPLAPSSKSTSGGTAALGCLVKDYFPEPVTVSWNSGALTSGVHTFPAVLQSSGLYSLSSVVTVPSSSLGTQTYICNVNHKPSNTKVDKRVEPKSCDKTHTCPPCPAPEAAGGPSVFLFPPKPKDTLMISRTPEVTCVVVDVSHEDPEVKFNWYVDGVEVHNAKTKPREEQYNSTYRVVSVLTVLHQDWLNGKEYKCKVSNKALGAPIEKTISKAKGQPREPQVYVYPPSREEMTKNQVSLTCLVKGFYPSDIAVEWESNGQPENNYKTTPPVLDSDGSFALVSKLTVDKSRWQQGNVFSCSVMHEALHNHYTQKSLSLSPGK

SEQ ID NO: 181 - protein, 690 aa, synthetic construct
  REGION 1..690: note = mSD15 + m3A7 mHc LALAPG
ITCPPPVSIEHADIRVKNYSVNSRERYVCNSGFKRKAGTSTLIECVINKNTNVAHWTTPSLKCIRDPALVHQRPAPPSGGSGGGGSGGGSGGGGSLQNWIDVRYDLEKIESLIQSIHIDTTLYTDSDFHPSCKVTAMNCFLLELQVILHEYSNMTLNETVRNVLYLANSTLSSNKNVAESGCKECEELEEKTFTEFLQSFIRIVQMFINTSGGGGSGGGGSGGGGSGGGGSGGGGSGGGGSQVQLVQSGAEVKKPGASVKVSCKASGHTFTSYYIHWVRQAPGQGLEWMGIINPSGGSTSYAQKFQGRVTMTRDTSTSTVYMELSSLRSEDTAVYYCARDRAYGGAGDYWGQGTLVTVSSAKTTAPSVYPLAPVCGDTTGSSVTLGCLVKGYFPEPVTLTWNSGSLSSGVHTFPAVLQSDLYTLSSSVTVTSSTWPSQSITCNVAHPASSTKVDKKIEPRGPTIKPCPPCKCPAPNAAGGPSVFIFPPKIKDVLMISLSPIVTCVVVDVSEDDPDVQISWFVNNVEVHTAQTQTHREDYNSTLRVVSALPIQHQDWMSGKEFKCKVNNKDLGAPIERTISKPKGSVRAPQVYVLPPPEEEMTKKQVTLTCMVTDFMPEDIYVEWTNNGKTELNYKNTEPVLDSDGSYFMYSKLRVEKKNWVERNSYSCSVVHEGLHNHHTTKSFSRTPGK

SEQ ID NO: 182 - protein, 690 aa, synthetic construct
  REGION 1..690: note = mSD15 + m3A7 mHc(T366L/ K392L/T394W) LALAPG
ITCPPPVSIEHADIRVKNYSVNSRERYVCNSGFKRKAGTSTLIECVINKNTNVAHWTTPSLKCIRDPALVHQRPAPPSGGSGGGGSGGGSGGGGSLQNWIDVRYDLEKIESLIQSIHIDTTLYTDSDFHPSCKVTAMNCFLLELQVILHEYSNMTLNETVRNVLYLANSTLSSNKNVAESGCKECEELEEKTFTEFLQSFIRIVQMFINTSGGGGSGGGGSGGGGSGGGGSGGGGSGGGGSQVQLVQSGAEVKKPGASVKVSCKASGHTFTSYYIHWVRQAPGQGLEWMGIINPSGGSTSYAQKFQGRVTMTRDTSTSTVYMELSSLRSEDTAVYYCARDRAYGGAGDYWGQGTLVTVSSAKTTAPSVYPLAPVCGDTTGSSVTLGCLVKGYFPEPVTLTWNSGSLSSGVHTFPAVLQSDLYTLSSSVTVTSSTWPSQSITCNVAHPASSTKVDKKIEPRGPTIKPCPPCKCPAPNAAGGPSVFIFPPKIKDVLMISLSPIVTCVVVDVSEDDPDVQISWFVNNVEVHTAQTQTHREDYNSTLRVVSALPIQHQDWMSGKEFKCKVNNKDLGAPIERTISKPKGSVRAPQVYVLPPPEEEMTKKQVTLLCMVTDFMPEDIYVEWTNNGKTELNYLNWEPVLDSDGSYFMYSKLRVEKKNWVERNSYSCSVVHEGLHNHHTTKSFSRTPGK

SEQ ID NO: 183 - protein, 658 aa, synthetic construct
  REGION 1..658: note = m3A7 mHc LALPG + mSD15
QVQLVQSGAEVKKPGASVKVSCKASGHTFTSYYIHWVRQAPGQGLEWMGIINPSGGSTSYAQKFQGRVTMTRDTSTSTVYMELSSLRSEDTAVYYCARDRAYGGAGDYWGQGTLVTVSSAKTTAPSVYPLAPVCGDTTGSSVTLGCLVKGYFPEPVTLTWNSGSLSSGVHTFPAVLQSDLYTLSSSVTVTSSTWPSQSITCNVAHPASSTKVDKKIEPRGPTIKPCPPCKCPAPNAAGGPSVFIFPPKIKDVLMISLSPIVTCVVVDVSEDDPDVQISWFVNNVEVHTAQTQTHREDYNSTLRVVSALPIQHQDWMSGKEFKCKVNNKDLGAPIERTISKPKGSVRAPQVYVLPPPEEEMTKKQVTLTCMVTDFMPEDIYVEWTNNGKTELNYKNTEPVLDSDGSYFMYSKLRVEKKNWVERNSYSCSVVHEGLHNHHTTKSFSRTPGSCPPPVSIEHADIRVKNYSVNSRERYVCNSGFKRKAGTSTLIECVINKNTNVAHWTTPSLKCIRDPALVHQRPAPPSGGSGGGGSGGGSGGGGSLQNWIDVRYDLEKIESLIQSIHIDTTLYTDSDFHPSCKVTAMNCFLLELQVILHEYSNMTLNETVRNVLYLANSTLSSNKNVAESGCKECEELEEKTFTEFLQSFIRIVQMFINTS

SEQ ID NO: 184 - protein, 658 aa, synthetic construct
  REGION 1..658: note = m3A7 mHC(T366L/K392L/T394W) + mSD15LALAPG
QVQLVQSGAEVKKPGASVKVSCKASGHTFTSYYIHWVRQAPGQGLEWMGIINPSGGSTSYAQKFQGRVTMTRDTSTSTVYMELSSLRSEDTAVYYCARDRAYGGAGDYWGQGTLVTVSSAKTTAPSVYPLAPVCGDTTGSSVTLGCLVKGYFPEPVTLTWNSGSLSSGVHTFPAVLQSDLYTLSSSVTVTSSTWPSQSITCNVAHPASSTKVDKKIEPRGPTIKPCPPCKCPAPNAAGGPSVFIFPPKIKDVLMISLSPIVTCVVVDVSEDDPDVQISWFVNNVEVHTAQTQTHREDYNSTLRVVSALPIQHQDWMSGKEFKCKVNNKDLGAPIERTISKPKGSVRAPQVYVLPPPEEEMTKKQVTLLCMVTDFMPEDIYVEWTNNGKTELNYLNWEPVLDSDGSYFMYSKLRVEKKNWVERNSYSCSVVHEGLHNHHTTKSFSRTPGSCPPPVSIEHADIRVKNYSVNSRERYVCNSGFKRKAGTSTLIECVINKNTNVAHWTTPSLKCIRDPALVHQRPAPPSGGSGGGGSGGGSGGGGSLQNWIDVRYDLEKIESLIQSIHIDTTLYTDSDFHPSCKVTAMNCFLLELQVILHEYSNMTLNETVRNVLYLANSTLSSNKNVAESGCKECEELEEKTFTEFLQSFIRIVQMFINTS

SEQ ID NO: 185 - protein, 445 aa, synthetic construct
  REGION 1..445: note = DP47 mHC (L351Y/F405A/Y407V) LALAPG
EVQLLESGGGLVQPGGSLRLSCAASGFTFSSYAMSWVRQAPGKGLEWVSAISGSGGSTYYADSVKGRFTISRDNSKNTLYLQMNSLRAEDTAVYYCAKGSGFDYWGQGTLVTVSSAKTTAPSVYPLAPVCGDTTGSSVTLGCLVKGYFPEPVTLTWNSGSLSSGVHTFPAVLQSDLYTLSSSVTVTSSTWPSQSITCNVAHPASSTKVDKKIEPRGPTIKPCPPCKCPAPNAAGGPSVFIFPPKIKDVLMISLSPIVTCVVVDVSEDDPDVQISWFVNNVEVHTAQTQTHREDYNSTLRVVSALPIQHQDWMSGKEFKCKVNNKDLGAPIERTISKPKGSVRAPQVYVYPPPEEEMTKKQVTLLCMVTDFMPEDIYVEWTNNGKTELNYKNTEPVLDSDGSYAMVSKLRVEKKNWVERNSYSCSVVHEGLHNHHTTKSFSRTPGK

SEQ ID NO: 186 - protein, 215 aa, synthetic construct
  REGION 1..215: note = DP47 mLC
EIVLTQSPGTLSLSPGERATLSCRASQSVSSSYLAWYQQKPGQAPRLLIYGASSRATGIPDRFSGSGSGTDFTLTISRLEPEDFAVYYCQQYGSSPLTFGQGTKVEIKRADAAPTVSIFPPSSEQLTSGGASVVCFLNNFYPKDINVKWKIDGSERQNGVLNSWTDQDSKDSTYSMSSTLTLTKDEYERHNSYTCEATHKTSTSPIVKSFNRNEC

SEQ ID NO: 187 - protein, 686 aa, synthetic construct
  REGION 1..686: note = mSD15 + DP47 mHC LALAPG
ITCPPPVSIEHADIRVKNYSVNSRERYVCNSGFKRKAGTSTLIECVINKNTNVAHWTTPSLKCIRDPALVHQRPAPPSGGSGGGGSGGGSGGGGSLQNWIDVRYDLEKIESLIQSIHIDTTLYTDSDFHPSCKVTAMNCFLLELQVILHEYSNMTLNETVRNVLYLANSTLSSNKNVAESGCKECEELEEKTFTEFLQSFIRIVQMFINTSGGGGSGGGGSGGGGSGGGGSGGGGSGGGGSEVQLLESGGGLVQPGGSLRLSCAASGFTFSSYAMSWVRQAPGKGLEWVSAISGSGGSTYYADSVKGRFTISRDNSKNTLYLQMNSLRAEDTAVYYCAKGSGFDYWGQGTLVTVSSAKTTAPSVYPLAPVCGDTTGSSVTLGCLVKGYFPEPVTLTWNSGSLSSGVHTFPAVLQSDLYTLSSSVTVTSSTWPSQSITCNVAHPASSTKVDKKIEPRGPTIKPCPPCKCPAPNAAGGPSVFIFPPKIKDVLMISLSPIVTCVVVDVSEDDPDVQISWFVNNVEVHTAQTQTHREDYNSTLRVVSALPIQHQDWMSGKEFKCKVNNKDLGAPIERTISKPKGSVRAPQVYVLPPPEEEMTKKQVTLTCMVTDFMPEDIYVEWTNNGKTELNYKNTEPVLDSDGSYFMYSKLRVEKKNWVERNSYSCSVVHEGLHNHHTTKSFSRTPGK

SEQ ID NO: 188 - protein, 686 aa, synthetic construct
  REGION 1..686: note = mSD15 + DP47 mHC (T366L/K392L/T394W)LALAPG
ITCPPPVSIEHADIRVKNYSVNSRERYVCNSGFKRKAGTSTLIECVINKNTNVAHWTTPSLKCIRDPALVHQRPAPPSGGSGGGGSGGGSGGGGSLQNWIDVRYDLEKIESLIQSIHIDTTLYTDSDFHPSCKVTAMNCFLLELQVILHEYSNMTLNETVRNVLYLANSTLSSNKNVAESGCKECEELEEKTFTEFLQSFIRIVQMFINTSGGGGSGGGGSGGGGSGGGGSGGGGSGGGGSEVQLLESGGGLVQPGGSLRLSCAASGFTFSSYAMSWVRQAPGKGLEWVSAISGSGGSTYYADSVKGRFTISRDNSKNTLYLQMNSLRAEDTAVYYCAKGSGFDYWGQGTLVTVSSAKTTAPSVYPLAPVCGDTTGSSVTLGCLVKGYFPEPVTLTWNSGSLSSGVHTFPAVLQSDLYTLSSSVTVTSSTWPSQSITCNVAHPASSTKVDKKIEPRGPTIKPCPPCKCPAPNAAGGPSVFIFPPKIKDVLMISLSPIVTCVVVDVSEDDPDVQISWFVNNVEVHTAQTQTHREDYNSTLRVVSALPIQHQDWMSGKEFKCKVNNKDLGAPIERTISKPKGSVRAPQVYVLPPPEEEMTKKQVTLLCMVTDFMPEDIYVEWTNNGKTELNYLNWEPVLDSDGSYFMYSKLRVEKKNWVERNSYSCSVVHEGLHNHHTTKSFSRTPGK

SEQ ID NO: 189 - protein, 654 aa, synthetic construct
  REGION 1..654: note = DP47 mHc LALAPG + mSD15
EVQLLESGGGLVQPGGSLRLSCAASGFTFSSYAMSWVRQAPGKGLEWVSAISGSGGSTYYADSVKGRFTISRDNSKNTLYLQMNSLRAEDTAVYYCAKGSGFDYWGQGTLVTVSSAKTTAPSVYPLAPVCGDTTGSSVTLGCLVKGYFPEPVTLTWNSGSLSSGVHTFPAVLQSDLYTLSSSVTVTSSTWPSQSITCNVAHPASSTKVDKKIEPRGPTIKPCPPCKCPAPNAAGGPSVFIFPPKIKDVLMISLSPIVTCVVVDVSEDDPDVQISWFVNNVEVHTAQTQTHREDYNSTLRVVSALPIQHQDWMSGKEFKCKVNNKDLGAPIERTISKPKGSVRAPQVYVLPPPEEEMTKKQVTLTCMVTDFMPEDIYVEWTNNGKTELNYKNTEPVLDSDGSYFMYSKLRVEKKNWVERNSYSCSVVHEGLHNHHTTKSFSRTPGSCPPPVSIEHADIRVKNYSVNSRERYVCNSGFKRKAGTSTLIECVINKNTNVAHWTTPSLKCIRDPALVHQRPAPPSGGSGGGGSGGGSGGGGSLQNWIDVRYDLEKIESLIQSIHIDTTLYTDSDFHPSCKVTAMNCFLLELQVILHEYSNMTLNETVRNVLYLANSTLSSNKNVAESGCKECEELEEKTFTEFLQSFIRIVQMFINTS

SEQ ID NO: 190 - protein, 654 aa, synthetic construct
  REGION 1..654: note = DP47 mHC (T366L/K392L/T394W) LALAPG + mSD15
EVQLLESGGGLVQPGGSLRLSCAASGFTFSSYAMSWVRQAPGKGLEWVSAISGSGGSTYYADSVKGRFTISRDNSKNTLYLQMNSLRAEDTAVYYCAKGSGFDYWGQGTLVTVSSAKTTAPSVYPLAPVCGDTTGSSVTLGCLVKGYFPEPVTLTWNSGSLSSGVHTFPAVLQSDLYTLSSSVTVTSSTWPSQSITCNVAHPASSTKVDKKIEPRGPTIKPCPPCKCPAPNAAGGPSVFIFPPKIKDVLMISLSPIVTCVVVDVSEDDPDVQISWFVNNVEVHTAQTQTHREDYNSTLRVVSALPIQHQDWMSGKEFKCKVNNKDLGAPIERTISKPKGSVRAPQVYVLPPPEEEMTKKQVTLLCMVTDFMPEDIYVEWTNNGKTELNYLNWEPVLDSDGSYFMYSKLRVEKKNWVERNSYSCSVVHEGLHNHHTTKSFSRTPGSCPPPVSIEHADIRVKNYSVNSRERYVCNSGFKRKAGTSTLIECVINKNTNVAHWTTPSLKCIRDPALVHQRPAPPSGGSGGGGSGGGSGGGGSLQNWIDVRYDLEKIESLIQSIHIDTTLYTDSDFHPSCKVTAMNCFLLELQVILHEYSNMTLNETVRNVLYLANSTLSSNKNVAESGCKECEELEEKTFTEFLQSFIRIVQMFINTS

SEQ ID NO: 191 - protein, 445 aa, synthetic construct
  REGION 1..445: note = DP47 HC (T350V/T366L/K392L/T394W) LALAPG
EVQLLESGGGLVQPGGSLRLSCAASGFTFSSYAMSWVRQAPGKGLEWVSAISGSGGSTYYADSVKGRFTISRDNSKNTLYLQMNSLRAEDTAVYYCAKGSGFDYWGQGTLVTVSSASTKGPSVFPLAPSSKSTSGGTAALGCLVKDYFPEPVTVSWNSGALTSGVHTFPAVLQSSGLYSLSSVVTVPSSSLGTQTYICNVNHKPSNTKVDKRVEPKSCDKTHTCPPCPAPEAAGGPSVFLFPPKPKDTLMISRTPEVTCVVVDVSHEDPEVKFNWYVDGVEVHNAKTKPREEQYNSTYRVVSVLTVLHQDWLNGKEYKCKVSNKALGAPIEKTISKAKGQPREPQVYVLPPSREEMTKNQVSLLCLVKGFYPSDIAVEWESNGQPENNYLTWPPVLDSDGSFFLYSKLTVDKSRWQQGNVFSCSVMHEALHNHYTQKSLSLSPGK

SEQ ID NO: 192 - protein, 215 aa, synthetic construct
  REGION 1..215: note = DP47 LC
EIVLTQSPGTLSLSPGERATLSCRASQSVSSSYLAWYQQKPGQAPRLLIYGASSRATGIPDRFSGSGSGTDFTLTISRLEPEDFAVYYCQQYGSSPLTFGQGTKVEIKRTVAAPSVFIFPPSDEQLKSGTASVVCLLNNFYPREAKVQWKVDNALQSGNSQESVTEQDSKDSTYSLSSTLTLSKADYEKHKVYACEVTHQGLSSPVTKSFNRGEC

SEQ ID NO: 193 - protein, 686 aa, synthetic construct
  REGION 1..686: note = hSD15 + DP47 HC LALPG
ITCPPPMSVEHADIWVKSYSLYSRERYICNSGFKRKAGTSSLTECVLNKATNVAHWTTPSLKCIRDPALVHQRPAPPSGGSGGGGSGGGSGGGGSLQNWVNVISDLKKIEDLIQSMHIDATLYTESDVHPSCKVTAMKCFLLELQVISLESGDASIHDTVENLIILANNSLSSNGNVTESGCKECEELEEKNIKEFLQSFVHIVQMFINTSGGGGSGGGGSGGGGSGGGGSGGGGSGGGGSEVQLLESGGGLVQPGGSLRLSCAASGFTFSSYAMSWVRQAPGKGLEWVSAISGSGGSTYYADSVKGRFTISRDNSKNTLYLQMNSLRAEDTAVYYCAKGSGFDYWGQGTLVTVSSASTKGPSVFPLAPSSKSTSGGTAALGCLVKDYFPEPVTVSWNSGALTSGVHTFPAVLQSSGLYSLSSVVTVPSSSLGTQTYICNVNHKPSNTKVDKRVEPKSCDKTHTCPPCPAPEAAGGPSVFLFPPKPKDTLMISRTPEVTCVVVDVSHEDPEVKFNWYVDGVEVHNAKTKPREEQYNSTYRVVSVLTVLHQDWLNGKEYKCKVSNKALGAPIEKTISKAKGQPREPQVYTLPPSREEMTKNQVSLTCLVKGFYPSDIAVEWESNGQPENNYKTTPPVLDSDGSFFLYSKLTVDKSRWQQGNVFSCSVMHEALHNHYTQKSLSLSPGK

SEQ ID NO: 194 - protein, 686 aa, synthetic construct
  REGION 1..686: note = hSD15 + DP47 HC (T350V/L351Y/F405A/Y407V) LALAPG
ITCPPPMSVEHADIWVKSYSLYSRERYICNSGFKRKAGTSSLTECVLNKATNVAHWTTPSLKCIRDPALVHQRPAPPSGGSGGGGSGGGSGGGGSLQNWVNVISDLKKIEDLIQSMHIDATLYTESDVHPSCKVTAMKCFLLELQVISLESGDASIHDTVENLIILANNSLSSNGNVTESGCKECEELEEKNIKEFLQSFVHIVQMFINTSGGGGSGGGGSGGGGSGGGGSGGGGSGGGGSEVQLLESGGGLVQPGGSLRLSCAASGFTFSSYAMSWVRQAPGKGLEWVSAISGSGGSTYYADSVKGRFTISRDNSKNTLYLQMNSLRAEDTAVYYCAKGSGFDYWGQGTLVTVSSASTKGPSVFPLAPSSKSTSGGTAALGCLVKDYFPEPVTVSWNSGALTSGVHTFPAVLQSSGLYSLSSVVTVPSSSLGTQTYICNVNHKPSNTKVDKRVEPKSCDKTHTCPPCPAPEAAGGPSVFLFPPKPKDTLMISRTPEVTCVVVDVSHEDPEVKFNWYVDGVEVHNAKTKPREEQYNSTYRVVSVLTVLHQDWLNGKEYKCKVSNKALGAPIEKTISKAKGQPREPQVYVYPPSREEMTKNQVSLTCLVKGFYPSDIAVEWESNGQPENNYKTTPPVLDSDGSFALVSKLTVDKSRWQQGNVFSCSVMHEALHNHYTQKSLSLSPGK

SEQ ID NO: 195 - protein, 654 aa, synthetic construct
  REGION 1..654: note = DP47 HC +LALAPG hSD15
EVQLLESGGGLVQPGGSLRLSCAASGFTFSSYAMSWVRQAPGKGLEWVSAISGSGGSTYYADSVKGRFTISRDNSKNTLYLQMNSLRAEDTAVYYCAKGSGFDYWGQGTLVTVSSASTKGPSVFPLAPSSKSTSGGTAALGCLVKDYFPEPVTVSWNSGALTSGVHTFPAVLQSSGLYSLSSVVTVPSSSLGTQTYICNVNHKPSNTKVDKRVEPKSCDKTHTCPPCPAPEAAGGPSVFLFPPKPKDTLMISRTPEVTCVVVDVSHEDPEVKFNWYVDGVEVHNAKTKPREEQYNSTYRVVSVLTVLHQDWLNGKEYKCKVSNKALGAPIEKTISKAKGQPREPQVYTLPPSREEMTKNQVSLTCLVKGFYPSDIAVEWESNGQPENNYKTTPPVLDSDGSFFLYSKLTVDKSRWQQGNVFSCSVMHEALHNHYTQKSLSLSPGSCPPPMSVEHADIWVKSYSLYSRERYICNSGFKRKAGTSSLTECVLNKATNVAHWTTPSLKCIRDPALVHQRPAPPSGGSGGGGSGGGSGGGGSLQNWVNVISDLKKIEDLIQSMHIDATLYTESDVHPSCKVTAMKCFLLELQVISLESGDASIHDTVENLIILANNSLSSNGNVTESGCKECEELEEKNIKEFLQSFVHIVQMFINTS

SEQ ID NO: 196 - protein, 654 aa, synthetic construct
  REGION 1..654: note = DP47 HC (T350V/L351Y/F405A/Y407V) LALAPG + hSD15
EVQLLESGGGLVQPGGSLRLSCAASGFTFSSYAMSWVRQAPGKGLEWVSAISGSGGSTYYADSVKGRFTISRDNSKNTLYLQMNSLRAEDTAVYYCAKGSGFDYWGQGTLVTVSSASTKGPSVFPLAPSSKSTSGGTAALGCLVKDYFPEPVTVSWNSGALTSGVHTFPAVLQSSGLYSLSSVVTVPSSSLGTQTYICNVNHKPSNTKVDKRVEPKSCDKTHTCPPCPAPEAAGGPSVFLFPPKPKDTLMISRTPEVTCVVVDVSHEDPEVKFNWYVDGVEVHNAKTKPREEQYNSTYRVVSVLTVLHQDWLNGKEYKCKVSNKALGAPIEKTISKAKGQPREPQVYVYPPSREEMTKNQVSLTCLVKGFYPSDIAVEWESNGQPENNYKTTPPVLDSDGSFALVSKLTVDKSRWQQGNVFSCSVMHEALHNHYTQKSLSLSPGSCPPPMSVEHADIWVKSYSLYSRERYICNSGFKRKAGTSSLTECVLNKATNVAHWTTPSLKCIRDPALVHQRPAPPSGGSGGGGSGGGSGGGGSLQNWVNVISDLKKIEDLIQSMHIDATLYTESDVHPSCKVTAMKCFLLELQVISLESGDASIHDTVENLIILANNSLSSNGNVTESGCKECEELEEKNIKEFLQSFVHIVQMFINTS

SEQ ID NO: 197 - protein, 686 aa, synthetic construct
  REGION 1..686: note = N65A-hSD15 + DP47 HC (T350V/L351Y/F405A/Y407V) LALAPG
ITCPPPMSVEHADIWVKSYSLYSRERYICNSGFKRKAGTSSLTECVLNKATNVAHWTTPSLKCIRDPALVHQRPAPPSGGSGGGGSGGGSGGGGSLQNWVNVISDLKKIEDLIQSMHIDATLYTESDVHPSCKVTAMKCFLLELQVISLESGDASIHDTVEALIILANNSLSSNGNVTESGCKECEELEEKNIKEFLQSFVHIVQMFINTSGGGGSGGGGSGGGGSGGGGSGGGGSGGGGSEVQLLESGGGLVQPGGSLRLSCAASGFTFSSYAMSWVRQAPGKGLEWVSAISGSGGSTYYADSVKGRFTISRDNSKNTLYLQMNSLRAEDTAVYYCAKGSGFDYWGQGTLVTVSSASTKGPSVFPLAPSSKSTSGGTAALGCLVKDYFPEPVTVSWNSGALTSGVHTFPAVLQSSGLYSLSSVVTVPSSSLGTQTYICNVNHKPSNTKVDKRVEPKSCDKTHTCPPCPAPEAAGGPSVFLFPPKPKDTLMISRTPEVTCVVVDVSHEDPEVKFNWYVDGVEVHNAKTKPREEQYNSTYRVVSVLTVLHQDWLNGKEYKCKVSNKALGAPIEKTISKAKGQPREPQVYVYPPSREEMTKNQVSLTCLVKGFYPSDIAVEWESNGQPENNYKTTPPVLDSDGSFALVSKLTVDKSRWQQGNVFSCSVMHEALHNHYTQKSLSLSPGK

SEQ ID NO: 198 - protein, 686 aa, synthetic construct
  REGION 1..686: note = N65D-hSD15 + DP47 HC (T350V/L351Y/F405A/Y407V) LALAPG
ITCPPPMSVEHADIWVKSYSLYSRERYICNSGFKRKAGTSSLTECVLNKATNVAHWTTPSLKCIRDPALVHQRPAPPSGGSGGGGSGGGSGGGGSLQNWVNVISDLKKIEDLIQSMHIDATLYTESDVHPSCKVTAMKCFLLELQVISLESGDASIHDTVEDLIILANNSLSSNGNVTESGCKECEELEEKNIKEFLQSFVHIVQMFINTSGGGGSGGGGSGGGGSGGGGSGGGGSGGGGSEVQLLESGGGLVQPGGSLRLSCAASGFTFSSYAMSWVRQAPGKGLEWVSAISGSGGSTYYADSVKGRFTISRDNSKNTLYLQMNSLRAEDTAVYYCAKGSGFDYWGQGTLVTVSSASTKGPSVFPLAPSSKSTSGGTAALGCLVKDYFPEPVTVSWNSGALTSGVHTFPAVLQSSGLYSLSSVVTVPSSSLGTQTYICNVNHKPSNTKVDKRVEPKSCDKTHTCPPCPAPEAAGGPSVFLFPPKPKDTLMISRTPEVTCVVVDVSHEDPEVKFNWYVDGVEVHNAKTKPREEQYNSTYRVVSVLTVLHQDWLNGKEYKCKVSNKALGAPIEKTISKAKGQPREPQVYVYPPSREEMTKNQVSLTCLVKGFYPSDIAVEWESNGQPENNYKTTPPVLDSDGSFALVSKLTVDKSRWQQGNVFSCSVMHEALHNHYTQKSLSLSPGK

SEQ ID NO: 199 - protein, 686 aa, synthetic construct
  REGION 1..686: note = N65S-hSD15 + DP47 HC (T350V/L351Y/F405A/Y407V) LALAPG
ITCPPPMSVEHADIWVKSYSLYSRERYICNSGFKRKAGTSSLTECVLNKATNVAHWTTPSLKCIRDPALVHQRPAPPSGGSGGGGSGGGSGGGGSLQNWVNVISDLKKIEDLIQSMHIDATLYTESDVHPSCKVTAMKCFLLELQVISLESGDASIHDTVESLIILANNSLSSNGNVTESGCKECEELEEKNIKEFLQSFVHIVQMFINTSGGGGSGGGGSGGGGSGGGGSGGGGSGGGGSEVQLLESGGGLVQPGGSLRLSCAASGFTFSSYAMSWVRQAPGKGLEWVSAISGSGGSTYYADSVKGRFTISRDNSKNTLYLQMNSLRAEDTAVYYCAKGSGFDYWGQGTLVTVSSASTKGPSVFPLAPSSKSTSGGTAALGCLVKDYFPEPVTVSWNSGALTSGVHTFPAVLQSSGLYSLSSVVTVPSSSLGTQTYICNVNHKPSNTKVDKRVEPKSCDKTHTCPPCPAPEAAGGPSVFLFPPKPKDTLMISRTPEVTCVVVDVSHEDPEVKFNWYVDGVEVHNAKTKPREEQYNSTYRVVSVLTVLHQDWLNGKEYKCKVSNKALGAPIEKTISKAKGQPREPQVYVYPPSREEMTKNQVSLTCLVKGFYPSDIAVEWESNGQPENNYKTTPPVLDSDGSFALVSKLTVDKSRWQQGNVFSCSVMHEALHNHYTQKSLSLSPGK

SEQ ID NO: 200 - protein, 120 aa, synthetic construct
  REGION 1..120: note = D7A8 VH
EVQLLESGGGLVQPGGSLRLSCAASGFTFSAYRMFWVRQAPGKGLEWVSSIYPSGGITFYADSVKGRFTISRDNSKNTLYLQMNSLRAEDTAIYYCARIKLGTVTTVDYWGQGTLVTVSS

SEQ ID NO: 201 - protein, 450 aa, synthetic construct
  REGION 1..450: note = D7A8 full length HC
EVQLLESGGGLVQPGGSLRLSCAASGFTFSAYRMFWVRQAPGKGLEWVSSIYPSGGITFYADSVKGRFTISRDNSKNTLYLQMNSLRAEDTAIYYCARIKLGTVTTVDYWGQGTLVTVSSASTKGPSVFPLAPSSKSTSGGTAALGCLVKDYFPEPVTVSWNSGALTSGVHTFPAVLQSSGLYSLSSVVTVPSSSLGTQTYICNVNHKPSNTKVDKRVEPKSCDKTHTCPPCPAPELLGGPSVFLFPPKPKDTLMISRTPEVTCVVVDVSHEDPEVKFNWYVDGVEVHNAKTKPREEQYNSTYRVVSVLTVLHQDWLNGKEYKCKVSNKALPAPIEKTISKAKGQPREPQVYTLPPSREEMTKNQVSLTCLVKGFYPSDIAVEWESNGQPENNYKTTPPVLDSDGSFFLYSKLTVDKSRWQQGNVFSCSVMHEALHNHYTQKSLSLSPGK

SEQ ID NO: 202 - protein, 450 aa, synthetic construct
  REGION 1..450: note = D7A8 HC (S354C/T366W) LALA
EVQLLESGGGLVQPGGSLRLSCAASGFTFSAYRMFWVRQAPGKGLEWVSSIYPSGGITFYADSVKGRFTISRDNSKNTLYLQMNSLRAEDTAIYYCARIKLGTVTTVDYWGQGTLVTVSSASTKGPSVFPLAPSSKSTSGGTAALGCLVKDYFPEPVTVSWNSGALTSGVHTFPAVLQSSGLYSLSSVVTVPSSSLGTQTYICNVNHKPSNTKVDKRVEPKSCDKTHTCPPCPAPEAAGGPSVFLFPPKPKDTLMISRTPEVTCVVVDVSHEDPEVKFNWYVDGVEVHNAKTKPREEQYNSTYRVVSVLTVLHQDWLNGKEYKCKVSNKALPAPIEKTISKAKGQPREPQVYTLPPCREEMTKNQVSLWCLVKGFYPSDIAVEWESNGQPENNYKTTPPVLDSDGSFFLYSKLTVDKSRWQQGNVFSCSVMHEALHNHYTQKSLSLSPGK

SEQ ID NO: 203 - protein, 450 aa, synthetic construct
  REGION 1..450: note = D7A8 HC (T350V/ T366L/ K392L/ T394W) LALA
EVQLLESGGGLVQPGGSLRLSCAASGFTFSAYRMFWVRQAPGKGLEWVSSIYPSGGITFYADSVKGRFTISRDNSKNTLYLQMNSLRAEDTAIYYCARIKLGTVTTVDYWGQGTLVTVSSASTKGPSVFPLAPSSKSTSGGTAALGCLVKDYFPEPVTVSWNSGALTSGVHTFPAVLQSSGLYSLSSVVTVPSSSLGTQTYICNVNHKPSNTKVDKRVEPKSCDKTHTCPPCPAPEAAGGPSVFLFPPKPKDTLMISRTPEVTCVVVDVSHEDPEVKFNWYVDGVEVHNAKTKPREEQYNSTYRVVSVLTVLHQDWLNGKEYKCKVSNKALPAPIEKTISKAKGQPREPQVYVLPPSREEMTKNQVSLLCLVKGFYPSDIAVEWESNGQPENNYLTWPPVLDSDGSFFLYSKLTVDKSRWQQGNVFSCSVMHEALHNHYTQKSLSLSPGK

SEQ ID NO: 204 - protein, 113 aa, synthetic construct
  REGION 1..113: note = D7A8 VL
QSALTQPASVSGSPGQSITISCTGTSSDVGAYNYVSWYQQHPGKAPKLMIYDVSNRPSGVSNRFSGSKSGNTASLTISGLQAEDEADYYCSSYTSSSTRVFGTGTKVTVLGQP

SEQ ID NO: 205 - protein, 216 aa, synthetic construct
  REGION 1..216: note = D7A8 full length LC
QSALTQPASVSGSPGQSITISCTGTSSDVGAYNYVSWYQQHPGKAPKLMIYDVSNRPSGVSNRFSGSKSGNTASLTISGLQAEDEADYYCSSYTSSSTRVFGTGTKVTVLGQPKANPTVTLFPPSSEELQANKATLVCLISDFYPGAVTVAWKADGSPVKAGVETTKPSKQSNNKYAASSYLSLTPEQWKSHRSYSCQVTHEGSTVEKTVAPTECS

SEQ ID NO: 206 - protein, 681 aa, synthetic construct
  REGION 1..681: note = hSD15 + D7A8 HC LALA
ITCPPPMSVEHADIWVKSYSLYSRERYICNSGFKRKAGTSSLTECVLNKATNVAHWTTPSLKCIRDPALVHQRPAPPSGGSGGGGSGGGSGGGGSLQNWVNVISDLKKIEDLIQSMHIDATLYTESDVHPSCKVTAMKCFLLELQVISLESGDASIHDTVENLIILANNSLSSNGNVTESGCKECEELEEKNIKEFLQSFVHIVQMFINTSGGGGSGGGGSGGGGSGGGGSEVQLLESGGGLVQPGGSLRLSCAASGFTFSAYRMFWVRQAPGKGLEWVSSIYPSGGITFYADSVKGRFTISRDNSKNTLYLQMNSLRAEDTAIYYCARIKLGTVTTVDYWGQGTLVTVSSASTKGPSVFPLAPSSKSTSGGTAALGCLVKDYFPEPVTVSWNSGALTSGVHTFPAVLQSSGLYSLSSVVTVPSSSLGTQTYICNVNHKPSNTKVDKRVEPKSCDKTHTCPPCPAPEAAGGPSVFLFPPKPKDTLMISRTPEVTCVVVDVSHEDPEVKFNWYVDGVEVHNAKTKPREEQYNSTYRVVSVLTVLHQDWLNGKEYKCKVSNKALPAPIEKTISKAKGQPREPQVYTLPPSREEMTKNQVSLTCLVKGFYPSDIAVEWESNGQPENNYKTTPPVLDSDGSFFLYSKLTVDKSRWQQGNVFSCSVMHEALHNHYTQKSLSLSPGK

SEQ ID NO: 207 - protein, 681 aa, synthetic construct
  REGION 1..681: note = hSD15 + D7A8HC (Y349C/T366S/L368A/Y407V) LALA
ITCPPPMSVEHADIWVKSYSLYSRERYICNSGFKRKAGTSSLTECVLNKATNVAHWTTPSLKCIRDPALVHQRPAPPSGGSGGGGSGGGSGGGGSLQNWVNVISDLKKIEDLIQSMHIDATLYTESDVHPSCKVTAMKCFLLELQVISLESGDASIHDTVENLIILANNSLSSNGNVTESGCKECEELEEKNIKEFLQSFVHIVQMFINTSGGGGSGGGGSGGGGSGGGGSEVQLLESGGGLVQPGGSLRLSCAASGFTFSAYRMFWVRQAPGKGLEWVSSIYPSGGITFYADSVKGRFTISRDNSKNTLYLQMNSLRAEDTAIYYCARIKLGTVTTVDYWGQGTLVTVSSASTKGPSVFPLAPSSKSTSGGTAALGCLVKDYFPEPVTVSWNSGALTSGVHTFPAVLQSSGLYSLSSVVTVPSSSLGTQTYICNVNHKPSNTKVDKRVEPKSCDKTHTCPPCPAPEAAGGPSVFLFPPKPKDTLMISRTPEVTCVVVDVSHEDPEVKFNWYVDGVEVHNAKTKPREEQYNSTYRVVSVLTVLHQDWLNGKEYKCKVSNKALPAPIEKTISKAKGQPREPQVCTLPPSREEMTKNQVSLSCAVKGFYPSDIAVEWESNGQPENNYKTTPPVLDSDGSFFLVSKLTVDKSRWQQGNVFSCSVMHEALHNHYTQKSLSLSPGK

SEQ ID NO: 208 - protein, 681 aa, synthetic construct
  REGION 1..681: note = hSD15 + D7A8HC (T350V/L351Y/F405A/Y407V) LALA
ITCPPPMSVEHADIWVKSYSLYSRERYICNSGFKRKAGTSSLTECVLNKATNVAHWTTPSLKCIRDPALVHQRPAPPSGGSGGGGSGGGSGGGGSLQNWVNVISDLKKIEDLIQSMHIDATLYTESDVHPSCKVTAMKCFLLELQVISLESGDASIHDTVENLIILANNSLSSNGNVTESGCKECEELEEKNIKEFLQSFVHIVQMFINTSGGGGSGGGGSGGGGSGGGGSEVQLLESGGGLVQPGGSLRLSCAASGFTFSAYRMFWVRQAPGKGLEWVSSIYPSGGITFYADSVKGRFTISRDNSKNTLYLQMNSLRAEDTAIYYCARIKLGTVTTVDYWGQGTLVTVSSASTKGPSVFPLAPSSKSTSGGTAALGCLVKDYFPEPVTVSWNSGALTSGVHTFPAVLQSSGLYSLSSVVTVPSSSLGTQTYICNVNHKPSNTKVDKRVEPKSCDKTHTCPPCPAPEAAGGPSVFLFPPKPKDTLMISRTPEVTCVVVDVSHEDPEVKFNWYVDGVEVHNAKTKPREEQYNSTYRVVSVLTVLHQDWLNGKEYKCKVSNKALPAPIEKTISKAKGQPREPQVYVYPPSREEMTKNQVSLTCLVKGFYPSDIAVEWESNGQPENNYKTTPPVLDSDGSFALVSKLTVDKSRWQQGNVFSCSVMHEALHNHYTQKSLSLSPGK

SEQ ID NO: 209 - protein, 659 aa, synthetic construct
  REGION 1..659: note = D7A8 HC LALA + hSD15
EVQLLESGGGLVQPGGSLRLSCAASGFTFSAYRMFWVRQAPGKGLEWVSSIYPSGGITFYADSVKGRFTISRDNSKNTLYLQMNSLRAEDTAIYYCARIKLGTVTTVDYWGQGTLVTVSSASTKGPSVFPLAPSSKSTSGGTAALGCLVKDYFPEPVTVSWNSGALTSGVHTFPAVLQSSGLYSLSSVVTVPSSSLGTQTYICNVNHKPSNTKVDKRVEPKSCDKTHTCPPCPAPEAAGGPSVFLFPPKPKDTLMISRTPEVTCVVVDVSHEDPEVKFNWYVDGVEVHNAKTKPREEQYNSTYRVVSVLTVLHQDWLNGKEYKCKVSNKALPAPIEKTISKAKGQPREPQVYTLPPSREEMTKNQVSLTCLVKGFYPSDIAVEWESNGQPENNYKTTPPVLDSDGSFFLYSKLTVDKSRWQQGNVFSCSVMHEALHNHYTQKSLSLSPGSCPPPMSVEHADIWVKSYSLYSRERYICNSGFKRKAGTSSLTECVLNKATNVAHWTTPSLKCIRDPALVHQRPAPPSGGSGGGGSGGGSGGGGSLQNWVNVISDLKKIEDLIQSMHIDATLYTESDVHPSCKVTAMKCFLLELQVISLESGDASIHDTVENLIILANNSLSSNGNVTESGCKECEELEEKNIKEFLQSFVHIVQMFINTS

SEQ ID NO: 210 - protein, 658 aa, synthetic construct
  REGION 1..658: note = D7A8 HC (Y349C/T366S/L368A/Y407V) LALA+ hSD15
EVQLLESGGGLVQPGGSLRLSCAASGFTFSAYRMFWVRQAPGKGLEWVSSIYPSGGITFYADSVKGRFTISRDNSKNTLYLQMNSLRAEDTAIYYCARIKLGTVTTVDYWGQGTLVTVSSASTKGPSVFPLAPSSKSTSGGTAALGCLVKDYFPEPVTVSWNSGALTSGVHTFPAVLQSSGLYSLSSVVTVPSSSLGTQTYICNVNHKPSNTKVDKRVEPKSCDKTHTCPPCPAPEAAGGPSVFLFPPKPKDTLMISRTPEVTCVVVDVSHEDPEVKFNWYVDGVEVHNAKTKPREEQYNSTYRVVSVLTVLHQDWLNGKEYKCKVSNKALPAPIEKTISKAKGQPREPQVCTLPPSREEMTKNQVSLSCAVKGFYPSDIAVEWESNGQPENNYKTTPPVLDSDGSFFLVSKLTVDKSRWQQGNVFSCSVMHEALHNHYTQKSLSLSPGCPPPMSVEHADIWVKSYSLYSRERYICNSGFKRKAGTSSLTECVLNKATNVAHWTTPSLKCIRDPALVHQRPAPPSGGSGGGGSGGGSGGGGSLQNWVNVISDLKKIEDLIQSMHIDATLYTESDVHPSCKVTAMKCFLLELQVISLESGDASIHDTVENLIILANNSLSSNGNVTESGCKECEELEEKNIKEFLQSFVHIVQMFINTS

SEQ ID NO: 211 - protein, 658 aa, synthetic construct
  REGION 1..658: note = D7A8 HC (T350V/L351Y/F405A/Y407V) LALA+ hSD15
EVQLLESGGGLVQPGGSLRLSCAASGFTFSAYRMFWVRQAPGKGLEWVSSIYPSGGITFYADSVKGRFTISRDNSKNTLYLQMNSLRAEDTAIYYCARIKLGTVTTVDYWGQGTLVTVSSASTKGPSVFPLAPSSKSTSGGTAALGCLVKDYFPEPVTVSWNSGALTSGVHTFPAVLQSSGLYSLSSVVTVPSSSLGTQTYICNVNHKPSNTKVDKRVEPKSCDKTHTCPPCPAPEAAGGPSVFLFPPKPKDTLMISRTPEVTCVVVDVSHEDPEVKFNWYVDGVEVHNAKTKPREEQYNSTYRVVSVLTVLHQDWLNGKEYKCKVSNKALPAPIEKTISKAKGQPREPQVYVYPPSREEMTKNQVSLTCLVKGFYPSDIAVEWESNGQPENNYKTTPPVLDSDGSFALVSKLTVDKSRWQQGNVFSCSVMHEALHNHYTQKSLSLSPGCPPPMSVEHADIWVKSYSLYSRERYICNSGFKRKAGTSSLTECVLNKATNVAHWTTPSLKCIRDPALVHQRPAPPSGGSGGGGSGGGSGGGGSLQNWVNVISDLKKIEDLIQSMHIDATLYTESDVHPSCKVTAMKCFLLELQVISLESGDASIHDTVENLIILANNSLSSNGNVTESGCKECEELEEKNIKEFLQSFVHIVQMFINTS

SEQ ID NO: 212 - protein, 114 aa, synthetic construct
  REGION 1..114: note = Human IL-15 (mature protein, residue N65 is in bold)
NWVNVISDLKKIEDLIQSMHIDATLYTESDVHPSCKVTAMKCFLLELQVISLESGDASIHDTVENLIILANNSLSSNGNVTESGCKECEELEEKNIKEFLQSFVHIVQMFINTS

SEQ ID NO: 213 - protein, 266 aa, synthetic construct
  REGION 1..266: note = Human IL-15 R alpha subunit (signal peptide is underlined, residue N60 is in bold)
MAPRRARGCRTLGLPALLLLLLLRPPATRGITCPPPMSVEHADIWVKSYSLYSRERYICNSGFKRKAGTSSLTECVLNKATNVAHWTTPSLKCIRDPALVHQRPAPPSTVTTAGVTPQPESLSPSGKEPAASSPSSNNTAATTAAIVPGSQLMPSKSPSTGTTEISSHESSHGTPSQTTAKNWELTASASHQPPGVYPQHSDTTVAISTSTVLLCGLSAVSLLACYLKSRQTPPLASVEMEAMEALPVTWGTSSRDEDLENCSHHL

SEQ ID NO: 214 - protein, 61 aa, synthetic construct
  REGION 1..61: note = IL-15R alpha sushi domain
CPPPMSVEHADIWVKSYSLYSRERYICNSGFKRKAGTSSLTECVLNKATNVAHWTTPSLKC

SEQ ID NO: 215 - protein, 34 aa, synthetic construct
  REGION 1..34: note = Linker 1
IRDPALVHQRPAPPSGGSGGGGSGGGSGGGGSLQ

SEQ ID NO: 216 - protein, 30 aa, synthetic construct
  REGION 1..30: note = Linker 2
GGGGSGGGGSGGGGSGGGGSGGGGSGGGGS

SEQ ID NO: 217 - protein, 34 aa, synthetic construct
  REGION 1..34: note = Exemplary linker
IRDPSGGGGSGGGGSGGGGSGGGGSGGGGSGGGG

SEQ ID NO: 218 - protein, 34 aa, synthetic construct
  REGION 1..34: note = Exemplary linker
IRDPGGGGSGGGGSGGGGSGGGGSGGGGSGGGGS

SEQ ID NO: 219 - protein, 214 aa, synthetic construct; identical to SEQ ID NO: 170
  REGION 1..214: note = 38B2 LC

SEQ ID NO: 220 - protein, 447 aa, synthetic construct
  REGION 1..447: note = 38B2 HC1-1 (T350V/T366L/K392L/T394W) LALAPG
EVQLLESGGGLVQPGGSLRLSCAASGFTFSSYWMSWVRQAPGKGLEWVSAISGSGGSTYYADSVKGRFTISRDNSKNTLYLQMNSLRAEDTAVYYCASSPLQWVDVWGQGTTVTVSSASTKGPSVFPLAPSSKSTSGGTAALGCLVKDYFPEPVTVSWNSGALTSGVHTFPAVLQSSGLYSLSSVVTVPSSSLGTQTYICNVNHKPSNTKVDKKVEPKSCDKTHTCPPCPAPEAAGGPSVFLFPPKPKDTLMISRTPEVTCVVVDVSHEDPEVKFNWYVDGVEVHNAKTKPREEQYNSTYRVVSVLTVLHQDWLNGKEYKCKVSNKALGAPIEKTISKAKGQPREPQVYVLPPSRDELTKNQVSLLCLVKGFYPSDIAVEWESNGQPENNYLTWPPVLDSDGSFFLYSKLTVDKSRWQQGNVFSCSVMHEALHNHYTQKSLSLSPGK

SEQ ID NO: 221 - protein, 447 aa, synthetic construct
  REGION 1..447: note = 38B2 HC1-2 (T350V/L351Y/F405A/Y407V) LALAPG
EVQLLESGGGLVQPGGSLRLSCAASGFTFSSYWMSWVRQAPGKGLEWVSAISGSGGSTYYADSVKGRFTISRDNSKNTLYLQMNSLRAEDTAVYYCASSPLQWVDVWGQGTTVTVSSASTKGPSVFPLAPSSKSTSGGTAALGCLVKDYFPEPVTVSWNSGALTSGVHTFPAVLQSSGLYSLSSVVTVPSSSLGTQTYICNVNHKPSNTKVDKKVEPKSCDKTHTCPPCPAPEAAGGPSVFLFPPKPKDTLMISRTPEVTCVVVDVSHEDPEVKFNWYVDGVEVHNAKTKPREEQYNSTYRVVSVLTVLHQDWLNGKEYKCKVSNKALGAPIEKTISKAKGQPREPQVYVYPPSRDELTKNQVSLTCLVKGFYPSDIAVEWESNGQPENNYKTTPPVLDSDGSFALVSKLTVDKSRWQQGNVFSCSVMHEALHNHYTQKSLSLSPGK

SEQ ID NO: 222 - protein, 447 aa, synthetic construct
  REGION 1..447: note = 38B2 HC1-3 (CW-CSAV) S354C/T366W LALAPG
EVQLLESGGGLVQPGGSLRLSCAASGFTFSSYWMSWVRQAPGKGLEWVSAISGSGGSTYYADSVKGRFTISRDNSKNTLYLQMNSLRAEDTAVYYCASSPLQWVDVWGQGTTVTVSSASTKGPSVFPLAPSSKSTSGGTAALGCLVKDYFPEPVTVSWNSGALTSGVHTFPAVLQSSGLYSLSSVVTVPSSSLGTQTYICNVNHKPSNTKVDKKVEPKSCDKTHTCPPCPAPEAAGGPSVFLFPPKPKDTLMISRTPEVTCVVVDVSHEDPEVKFNWYVDGVEVHNAKTKPREEQYNSTYRVVSVLTVLHQDWLNGKEYKCKVSNKALGAPIEKTISKAKGQPREPQVYTLPPCRDELTKNQVSLWCLVKGFYPSDIAVEWESNGQPENNYKTTPPVLDSDGSFFLYSKLTVDKSRWQQGNVFSCSVMHEALHNHYTQKSLSLSPGK

SEQ ID NO: 223 - protein, 447 aa, synthetic construct
  REGION 1..447: note = 38B2 HC1-4(CW-CSAV) Y349C/T366S/L368A/Y407V LALAPG
EVQLLESGGGLVQPGGSLRLSCAASGFTFSSYWMSWVRQAPGKGLEWVSAISGSGGSTYYADSVKGRFTISRDNSKNTLYLQMNSLRAEDTAVYYCASSPLQWVDVWGQGTTVTVSSASTKGPSVFPLAPSSKSTSGGTAALGCLVKDYFPEPVTVSWNSGALTSGVHTFPAVLQSSGLYSLSSVVTVPSSSLGTQTYICNVNHKPSNTKVDKKVEPKSCDKTHTCPPCPAPEAAGGPSVFLFPPKPKDTLMISRTPEVTCVVVDVSHEDPEVKFNWYVDGVEVHNAKTKPREEQYNSTYRVVSVLTVLHQDWLNGKEYKCKVSNKALGAPIEKTISKAKGQPREPQVCTLPPSRDELTKNQVSLSCAVKGFYPSDIAVEWESNGQPENNYKTTPPVLDSDGSFFLVSKLTVDKSRWQQGNVFSCSVMHEALHNHYTQKSLSLSPGK

SEQ ID NO: 224 - protein, 688 aa, synthetic construct
  REGION 1..688: note = 65N-38B2 HC2-1 (T350V/L351Y/F405A/Y407V) LALAPG
ITCPPPMSVEHADIWVKSYSLYSRERYICNSGFKRKAGTSSLTECVLNKATNVAHWTTPSLKCIRDPALVHQRPAPPSGGSGGGGSGGGSGGGGSLQNWVNVISDLKKIEDLIQSMHIDATLYTESDVHPSCKVTAMKCFLLELQVISLESGDASIHDTVENLIILANNSLSSNGNVTESGCKECEELEEKNIKEFLQSFVHIVQMFINTSGGGGSGGGGSGGGGSGGGGSGGGGSGGGGSEVQLLESGGGLVQPGGSLRLSCAASGFTFSSYWMSWVRQAPGKGLEWVSAISGSGGSTYYADSVKGRFTISRDNSKNTLYLQMNSLRAEDTAVYYCASSPLQWVDVWGQGTTVTVSSASTKGPSVFPLAPSSKSTSGGTAALGCLVKDYFPEPVTVSWNSGALTSGVHTFPAVLQSSGLYSLSSVVTVPSSSLGTQTYICNVNHKPSNTKVDKKVEPKSCDKTHTCPPCPAPEAAGGPSVFLFPPKPKDTLMISRTPEVTCVVVDVSHEDPEVKFNWYVDGVEVHNAKTKPREEQYNSTYRVVSVLTVLHQDWLNGKEYKCKVSNKALGAPIEKTISKAKGQPREPQVYVYPPSRDELTKNQVSLTCLVKGFYPSDIAVEWESNGQPENNYKTTPPVLDSDGSFALVSKLTVDKSRWQQGNVFSCSVMHEALHNHYTQKSLSLSPGK

SEQ ID NO: 225 - protein, 688 aa, synthetic construct
  REGION 1..688: note = 65N-38B2 HC2-2(T350V/ T366L/K392L/T394W) LALAPG
ITCPPPMSVEHADIWVKSYSLYSRERYICNSGFKRKAGTSSLTECVLNKATNVAHWTTPSLKCIRDPALVHQRPAPPSGGSGGGGSGGGSGGGGSLQNWVNVISDLKKIEDLIQSMHIDATLYTESDVHPSCKVTAMKCFLLELQVISLESGDASIHDTVENLIILANNSLSSNGNVTESGCKECEELEEKNIKEFLQSFVHIVQMFINTSGGGGSGGGGSGGGGSGGGGSGGGGSGGGGSEVQLLESGGGLVQPGGSLRLSCAASGFTFSSYWMSWVRQAPGKGLEWVSAISGSGGSTYYADSVKGRFTISRDNSKNTLYLQMNSLRAEDTAVYYCASSPLQWVDVWGQGTTVTVSSASTKGPSVFPLAPSSKSTSGGTAALGCLVKDYFPEPVTVSWNSGALTSGVHTFPAVLQSSGLYSLSSVVTVPSSSLGTQTYICNVNHKPSNTKVDKKVEPKSCDKTHTCPPCPAPEAAGGPSVFLFPPKPKDTLMISRTPEVTCVVVDVSHEDPEVKFNWYVDGVEVHNAKTKPREEQYNSTYRVVSVLTVLHQDWLNGKEYKCKVSNKALGAPIEKTISKAKGQPREPQVYVLPPSRDELTKNQVSLLCLVKGFYPSDIAVEWESNGQPENNYLTWPPVLDSDGSFFLYSKLTVDKSRWQQGNVFSCSVMHEALHNHYTQKSLSLSPGK

SEQ ID NO: 226 - protein, 688 aa, synthetic construct
  REGION 1..688: note = 65N-38B2 HC2-3(CW-CSAV) Y349C/T366S/L368A/Y407V LALAPG
ITCPPPMSVEHADIWVKSYSLYSRERYICNSGFKRKAGTSSLTECVLNKATNVAHWTTPSLKCIRDPALVHQRPAPPSGGSGGGGSGGGSGGGGSLQNWVNVISDLKKIEDLIQSMHIDATLYTESDVHPSCKVTAMKCFLLELQVISLESGDASIHDTVENLIILANNSLSSNGNVTESGCKECEELEEKNIKEFLQSFVHIVQMFINTSGGGGSGGGGSGGGGSGGGGSGGGGSGGGGSEVQLLESGGGLVQPGGSLRLSCAASGFTFSSYWMSWVRQAPGKGLEWVSAISGSGGSTYYADSVKGRFTISRDNSKNTLYLQMNSLRAEDTAVYYCASSPLQWVDVWGQGTTVTVSSASTKGPSVFPLAPSSKSTSGGTAALGCLVKDYFPEPVTVSWNSGALTSGVHTFPAVLQSSGLYSLSSVVTVPSSSLGTQTYICNVNHKPSNTKVDKKVEPKSCDKTHTCPPCPAPEAAGGPSVFLFPPKPKDTLMISRTPEVTCVVVDVSHEDPEVKFNWYVDGVEVHNAKTKPREEQYNSTYRVVSVLTVLHQDWLNGKEYKCKVSNKALGAPIEKTISKAKGQPREPQVCTLPPSRDELTKNQVSLSCAVKGFYPSDIAVEWESNGQPENNYKTTPPVLDSDGSFFLVSKLTVDKSRWQQGNVFSCSVMHEALHNHYTQKSLSLSPGK

SEQ ID NO: 227 - protein, 688 aa, synthetic construct
  REGION 1..688: note = 65N-38B2 HC2-4 S354C/T366W LALAPG
ITCPPPMSVEHADIWVKSYSLYSRERYICNSGFKRKAGTSSLTECVLNKATNVAHWTTPSLKCIRDPALVHQRPAPPSGGSGGGGSGGGSGGGGSLQNWVNVISDLKKIEDLIQSMHIDATLYTESDVHPSCKVTAMKCFLLELQVISLESGDASIHDTVENLIILANNSLSSNGNVTESGCKECEELEEKNIKEFLQSFVHIVQMFINTSGGGGSGGGGSGGGGSGGGGSGGGGSGGGGSEVQLLESGGGLVQPGGSLRLSCAASGFTFSSYWMSWVRQAPGKGLEWVSAISGSGGSTYYADSVKGRFTISRDNSKNTLYLQMNSLRAEDTAVYYCASSPLQWVDVWGQGTTVTVSSASTKGPSVFPLAPSSKSTSGGTAALGCLVKDYFPEPVTVSWNSGALTSGVHTFPAVLQSSGLYSLSSVVTVPSSSLGTQTYICNVNHKPSNTKVDKKVEPKSCDKTHTCPPCPAPEAAGGPSVFLFPPKPKDTLMISRTPEVTCVVVDVSHEDPEVKFNWYVDGVEVHNAKTKPREEQYNSTYRVVSVLTVLHQDWLNGKEYKCKVSNKALGAPIEKTISKAKGQPREPQVYTLPPCRDELTKNQVSLWCLVKGFYPSDIAVEWESNGQPENNYKTTPPVLDSDGSFFLYSKLTVDKSRWQQGNVFSCSVMHEALHNHYTQKSLSLSPGK

SEQ ID NO: 228 - protein, 688 aa, synthetic construct
  REGION 1..688: note = 65S-38B2 HC2-1(T350V/L351Y/F405A/Y407V) LALAPG
ITCPPPMSVEHADIWVKSYSLYSRERYICNSGFKRKAGTSSLTECVLNKATNVAHWTTPSLKCIRDPALVHQRPAPPSGGSGGGGSGGGSGGGGSLQNWVNVISDLKKIEDLIQSMHIDATLYTESDVHPSCKVTAMKCFLLELQVISLESGDASIHDTVESLIILANNSLSSNGNVTESGCKECEELEEKNIKEFLQSFVHIVQMFINTSGGGGSGGGGSGGGGSGGGGSGGGGSGGGGSEVQLLESGGGLVQPGGSLRLSCAASGFTFSSYWMSWVRQAPGKGLEWVSAISGSGGSTYYADSVKGRFTISRDNSKNTLYLQMNSLRAEDTAVYYCASSPLQWVDVWGQGTTVTVSSASTKGPSVFPLAPSSKSTSGGTAALGCLVKDYFPEPVTVSWNSGALTSGVHTFPAVLQSSGLYSLSSVVTVPSSSLGTQTYICNVNHKPSNTKVDKKVEPKSCDKTHTCPPCPAPEAAGGPSVFLFPPKPKDTLMISRTPEVTCVVVDVSHEDPEVKFNWYVDGVEVHNAKTKPREEQYNSTYRVVSVLTVLHQDWLNGKEYKCKVSNKALGAPIEKTISKAKGQPREPQVYVYPPSRDELTKNQVSLTCLVKGFYPSDIAVEWESNGQPENNYKTTPPVLDSDGSFALVSKLTVDKSRWQQGNVFSCSVMHEALHNHYTQKSLSLSPGK

SEQ ID NO: 229 - protein, 688 aa, synthetic construct
  REGION 1..688: note = 65S-38B2 HC2-2(T350V/T366L/K392L/T394W) LALAPG
ITCPPPMSVEHADIWVKSYSLYSRERYICNSGFKRKAGTSSLTECVLNKATNVAHWTTPSLKCIRDPALVHQRPAPPSGGSGGGGSGGGSGGGGSLQNWVNVISDLKKIEDLIQSMHIDATLYTESDVHPSCKVTAMKCFLLELQVISLESGDASIHDTVESLIILANNSLSSNGNVTESGCKECEELEEKNIKEFLQSFVHIVQMFINTSGGGGSGGGGSGGGGSGGGGSGGGGSGGGGSEVQLLESGGGLVQPGGSLRLSCAASGFTFSSYWMSWVRQAPGKGLEWVSAISGSGGSTYYADSVKGRFTISRDNSKNTLYLQMNSLRAEDTAVYYCASSPLQWVDVWGQGTTVTVSSASTKGPSVFPLAPSSKSTSGGTAALGCLVKDYFPEPVTVSWNSGALTSGVHTFPAVLQSSGLYSLSSVVTVPSSSLGTQTYICNVNHKPSNTKVDKKVEPKSCDKTHTCPPCPAPEAAGGPSVFLFPPKPKDTLMISRTPEVTCVVVDVSHEDPEVKFNWYVDGVEVHNAKTKPREEQYNSTYRVVSVLTVLHQDWLNGKEYKCKVSNKALGAPIEKTISKAKGQPREPQVYVLPPSRDELTKNQVSLLCLVKGFYPSDIAVEWESNGQPENNYLTWPPVLDSDGSFFLYSKLTVDKSRWQQGNVFSCSVMHEALHNHYTQKSLSLSPGK

SEQ ID NO: 230 - protein, 688 aa, synthetic construct
  REGION 1..688: note = 65S-38B2 HC2-3(CW-CSAV) Y349C/T366S/L368A/Y407V LALAP
ITCPPPMSVEHADIWVKSYSLYSRERYICNSGFKRKAGTSSLTECVLNKATNVAHWTTPSLKCIRDPALVHQRPAPPSGGSGGGGSGGGSGGGGSLQNWVNVISDLKKIEDLIQSMHIDATLYTESDVHPSCKVTAMKCFLLELQVISLESGDASIHDTVESLIILANNSLSSNGNVTESGCKECEELEEKNIKEFLQSFVHIVQMFINTSGGGGSGGGGSGGGGSGGGGSGGGGSGGGGSEVQLLESGGGLVQPGGSLRLSCAASGFTFSSYWMSWVRQAPGKGLEWVSAISGSGGSTYYADSVKGRFTISRDNSKNTLYLQMNSLRAEDTAVYYCASSPLQWVDVWGQGTTVTVSSASTKGPSVFPLAPSSKSTSGGTAALGCLVKDYFPEPVTVSWNSGALTSGVHTFPAVLQSSGLYSLSSVVTVPSSSLGTQTYICNVNHKPSNTKVDKKVEPKSCDKTHTCPPCPAPEAAGGPSVFLFPPKPKDTLMISRTPEVTCVVVDVSHEDPEVKFNWYVDGVEVHNAKTKPREEQYNSTYRVVSVLTVLHQDWLNGKEYKCKVSNKALGAPIEKTISKAKGQPREPQVCTLPPSRDELTKNQVSLSCAVKGFYPSDIAVEWESNGQPENNYKTTPPVLDSDGSFFLVSKLTVDKSRWQQGNVFSCSVMHEALHNHYTQKSLSLSPGK

SEQ ID NO: 231 - protein, 688 aa, synthetic construct
  REGION 1..688: note = 65S-38B2 HC2-4 S354C/T366W LALAPG
ITCPPPMSVEHADIWVKSYSLYSRERYICNSGFKRKAGTSSLTECVLNKATNVAHWTTPSLKCIRDPALVHQRPAPPSGGSGGGGSGGGSGGGGSLQNWVNVISDLKKIEDLIQSMHIDATLYTESDVHPSCKVTAMKCFLLELQVISLESGDASIHDTVESLIILANNSLSSNGNVTESGCKECEELEEKNIKEFLQSFVHIVQMFINTSGGGGSGGGGSGGGGSGGGGSGGGGSGGGGSEVQLLESGGGLVQPGGSLRLSCAASGFTFSSYWMSWVRQAPGKGLEWVSAISGSGGSTYYADSVKGRFTISRDNSKNTLYLQMNSLRAEDTAVYYCASSPLQWVDVWGQGTTVTVSSASTKGPSVFPLAPSSKSTSGGTAALGCLVKDYFPEPVTVSWNSGALTSGVHTFPAVLQSSGLYSLSSVVTVPSSSLGTQTYICNVNHKPSNTKVDKKVEPKSCDKTHTCPPCPAPEAAGGPSVFLFPPKPKDTLMISRTPEVTCVVVDVSHEDPEVKFNWYVDGVEVHNAKTKPREEQYNSTYRVVSVLTVLHQDWLNGKEYKCKVSNKALGAPIEKTISKAKGQPREPQVYTLPPCRDELTKNQVSLWCLVKGFYPSDIAVEWESNGQPENNYKTTPPVLDSDGSFFLYSKLTVDKSRWQQGNVFSCSVMHEALHNHYTQKSLSLSPGK

SEQ ID NO: 232 - protein, 688 aa, synthetic construct
  REGION 1..688: note = 65D-38B2 HC2-1(T350V/L351Y/F405A/Y407V) LALAPG
ITCPPPMSVEHADIWVKSYSLYSRERYICNSGFKRKAGTSSLTECVLNKATNVAHWTTPSLKCIRDPALVHQRPAPPSGGSGGGGSGGGSGGGGSLQNWVNVISDLKKIEDLIQSMHIDATLYTESDVHPSCKVTAMKCFLLELQVISLESGDASIHDTVEDLIILANNSLSSNGNVTESGCKECEELEEKNIKEFLQSFVHIVQMFINTSGGGGSGGGGSGGGGSGGGGSGGGGSGGGGSEVQLLESGGGLVQPGGSLRLSCAASGFTFSSYWMSWVRQAPGKGLEWVSAISGSGGSTYYADSVKGRFTISRDNSKNTLYLQMNSLRAEDTAVYYCASSPLQWVDVWGQGTTVTVSSASTKGPSVFPLAPSSKSTSGGTAALGCLVKDYFPEPVTVSWNSGALTSGVHTFPAVLQSSGLYSLSSVVTVPSSSLGTQTYICNVNHKPSNTKVDKKVEPKSCDKTHTCPPCPAPEAAGGPSVFLFPPKPKDTLMISRTPEVTCVVVDVSHEDPEVKFNWYVDGVEVHNAKTKPREEQYNSTYRVVSVLTVLHQDWLNGKEYKCKVSNKALGAPIEKTISKAKGQPREPQVYVYPPSRDELTKNQVSLTCLVKGFYPSDIAVEWESNGQPENNYKTTPPVLDSDGSFALVSKLTVDKSRWQQGNVFSCSVMHEALHNHYTQKSLSLSPGK

SEQ ID NO: 233 - protein, 688 aa, synthetic construct
  REGION 1..688: note = 65D-38B2 HC2-2(T350V/T366L/K392L/T394W) LALAPG
ITCPPPMSVEHADIWVKSYSLYSRERYICNSGFKRKAGTSSLTECVLNKATNVAHWTTPSLKCIRDPALVHQRPAPPSGGSGGGGSGGGSGGGGSLQNWVNVISDLKKIEDLIQSMHIDATLYTESDVHPSCKVTAMKCFLLELQVISLESGDASIHDTVEDLIILANNSLSSNGNVTESGCKECEELEEKNIKEFLQSFVHIVQMFINTSGGGGSGGGGSGGGGSGGGGSGGGGSGGGGSEVQLLESGGGLVQPGGSLRLSCAASGFTFSSYWMSWVRQAPGKGLEWVSAISGSGGSTYYADSVKGRFTISRDNSKNTLYLQMNSLRAEDTAVYYCASSPLQWVDVWGQGTTVTVSSASTKGPSVFPLAPSSKSTSGGTAALGCLVKDYFPEPVTVSWNSGALTSGVHTFPAVLQSSGLYSLSSVVTVPSSSLGTQTYICNVNHKPSNTKVDKKVEPKSCDKTHTCPPCPAPEAAGGPSVFLFPPKPKDTLMISRTPEVTCVVVDVSHEDPEVKFNWYVDGVEVHNAKTKPREEQYNSTYRVVSVLTVLHQDWLNGKEYKCKVSNKALGAPIEKTISKAKGQPREPQVYVLPPSRDELTKNQVSLLCLVKGFYPSDIAVEWESNGQPENNYLTWPPVLDSDGSFFLYSKLTVDKSRWQQGNVFSCSVMHEALHNHYTQKSLSLSPGK

SEQ ID NO: 234 - protein, 688 aa, synthetic construct
  REGION 1..688: note = 65D-38B2 HC2-3(CW-CSAV) Y349C/T366S/L368A/Y407V LALAPG
ITCPPPMSVEHADIWVKSYSLYSRERYICNSGFKRKAGTSSLTECVLNKATNVAHWTTPSLKCIRDPALVHQRPAPPSGGSGGGGSGGGSGGGGSLQNWVNVISDLKKIEDLIQSMHIDATLYTESDVHPSCKVTAMKCFLLELQVISLESGDASIHDTVEDLIILANNSLSSNGNVTESGCKECEELEEKNIKEFLQSFVHIVQMFINTSGGGGSGGGGSGGGGSGGGGSGGGGSGGGGSEVQLLESGGGLVQPGGSLRLSCAASGFTFSSYWMSWVRQAPGKGLEWVSAISGSGGSTYYADSVKGRFTISRDNSKNTLYLQMNSLRAEDTAVYYCASSPLQWVDVWGQGTTVTVSSASTKGPSVFPLAPSSKSTSGGTAALGCLVKDYFPEPVTVSWNSGALTSGVHTFPAVLQSSGLYSLSSVVTVPSSSLGTQTYICNVNHKPSNTKVDKKVEPKSCDKTHTCPPCPAPEAAGGPSVFLFPPKPKDTLMISRTPEVTCVVVDVSHEDPEVKFNWYVDGVEVHNAKTKPREEQYNSTYRVVSVLTVLHQDWLNGKEYKCKVSNKALGAPIEKTISKAKGQPREPQVCTLPPSRDELTKNQVSLSCAVKGFYPSDIAVEWESNGQPENNYKTTPPVLDSDGSFFLVSKLTVDKSRWQQGNVFSCSVMHEALHNHYTQKSLSLSPGK

SEQ ID NO: 235 - protein, 688 aa, synthetic construct
  REGION 1..688: note = 65D-38B2 HC2-4 S354C/T366W LALAPG
ITCPPPMSVEHADIWVKSYSLYSRERYICNSGFKRKAGTSSLTECVLNKATNVAHWTTPSLKCIRDPALVHQRPAPPSGGSGGGGSGGGSGGGGSLQNWVNVISDLKKIEDLIQSMHIDATLYTESDVHPSCKVTAMKCFLLELQVISLESGDASIHDTVEDLIILANNSLSSNGNVTESGCKECEELEEKNIKEFLQSFVHIVQMFINTSGGGGSGGGGSGGGGSGGGGSGGGGSGGGGSEVQLLESGGGLVQPGGSLRLSCAASGFTFSSYWMSWVRQAPGKGLEWVSAISGSGGSTYYADSVKGRFTISRDNSKNTLYLQMNSLRAEDTAVYYCASSPLQWVDVWGQGTTVTVSSASTKGPSVFPLAPSSKSTSGGTAALGCLVKDYFPEPVTVSWNSGALTSGVHTFPAVLQSSGLYSLSSVVTVPSSSLGTQTYICNVNHKPSNTKVDKKVEPKSCDKTHTCPPCPAPEAAGGPSVFLFPPKPKDTLMISRTPEVTCVVVDVSHEDPEVKFNWYVDGVEVHNAKTKPREEQYNSTYRVVSVLTVLHQDWLNGKEYKCKVSNKALGAPIEKTISKAKGQPREPQVYTLPPCRDELTKNQVSLWCLVKGFYPSDIAVEWESNGQPENNYKTTPPVLDSDGSFFLYSKLTVDKSRWQQGNVFSCSVMHEALHNHYTQKSLSLSPGK

SEQ ID NO: 236 - protein, 688 aa, synthetic construct
  REGION 1..688: note = 65S-38B2 HC2-5(T350V/L351Y/F405A/Y407V) LALAPG
ITCPPPMSVEHADIWVKSYSLYSRERYICNSGFKRKAGTSSLTECVLNKATNVAHWTTPSLKCIRDPALVHQRPAPPSGGGGSGGGGSGGGSGGGGSNWVNVISDLKKIEDLIQSMHIDATLYTESDVHPSCKVTAMKCFLLELQVISLESGDASIHDTVESLIILANNSLSSNGNVTESGCKECEELEEKNIKEFLQSFVHIVQMFINTSGGGGSGGGGSGGGGSGGGGSGGGGSGGGGSEVQLLESGGGLVQPGGSLRLSCAASGFTFSSYWMSWVRQAPGKGLEWVSAISGSGGSTYYADSVKGRFTISRDNSKNTLYLQMNSLRAEDTAVYYCASSPLQWVDVWGQGTTVTVSSASTKGPSVFPLAPSSKSTSGGTAALGCLVKDYFPEPVTVSWNSGALTSGVHTFPAVLQSSGLYSLSSVVTVPSSSLGTQTYICNVNHKPSNTKVDKKVEPKSCDKTHTCPPCPAPEAAGGPSVFLFPPKPKDTLMISRTPEVTCVVVDVSHEDPEVKFNWYVDGVEVHNAKTKPREEQYNSTYRVVSVLTVLHQDWLNGKEYKCKVSNKALGAPIEKTISKAKGQPREPQVYVYPPSRDELTKNQVSLTCLVKGFYPSDIAVEWESNGQPENNYKTTPPVLDSDGSFALVSKLTVDKSRWQQGNVFSCSVMHEALHNHYTQKSLSLSPGK

SEQ ID NO: 237 - protein, 688 aa, synthetic construct
  REGION 1..688: note = 65S-38B2 HC2-6(T350V/T366L/K392L/T394W) LALAPG
ITCPPPMSVEHADIWVKSYSLYSRERYICNSGFKRKAGTSSLTECVLNKATNVAHWTTPSLKCIRDPALVHQRPAPPSGGGGSGGGGSGGGSGGGGSNWVNVISDLKKIEDLIQSMHIDATLYTESDVHPSCKVTAMKCFLLELQVISLESGDASIHDTVESLIILANNSLSSNGNVTESGCKECEELEEKNIKEFLQSFVHIVQMFINTSGGGGSGGGGSGGGGSGGGGSGGGGSGGGGSEVQLLESGGGLVQPGGSLRLSCAASGFTFSSYWMSWVRQAPGKGLEWVSAISGSGGSTYYADSVKGRFTISRDNSKNTLYLQMNSLRAEDTAVYYCASSPLQWVDVWGQGTTVTVSSASTKGPSVFPLAPSSKSTSGGTAALGCLVKDYFPEPVTVSWNSGALTSGVHTFPAVLQSSGLYSLSSVVTVPSSSLGTQTYICNVNHKPSNTKVDKKVEPKSCDKTHTCPPCPAPEAAGGPSVFLFPPKPKDTLMISRTPEVTCVVVDVSHEDPEVKFNWYVDGVEVHNAKTKPREEQYNSTYRVVSVLTVLHQDWLNGKEYKCKVSNKALGAPIEKTISKAKGQPREPQVYVLPPSRDELTKNQVSLLCLVKGFYPSDIAVEWESNGQPENNYLTWPPVLDSDGSFFLYSKLTVDKSRWQQGNVFSCSVMHEALHNHYTQKSLSLSPGK

SEQ ID NO: 238 - protein, 688 aa, synthetic construct
  REGION 1..688: note = 65S-38B2 HC2-7(CW-CSAV) Y349C/T366S/L368A/Y407V LALAPG
ITCPPPMSVEHADIWVKSYSLYSRERYICNSGFKRKAGTSSLTECVLNKATNVAHWTTPSLKCIRDPALVHQRPAPPSGGGGSGGGGSGGGSGGGGSNWVNVISDLKKIEDLIQSMHIDATLYTESDVHPSCKVTAMKCFLLELQVISLESGDASIHDTVESLIILANNSLSSNGNVTESGCKECEELEEKNIKEFLQSFVHIVQMFINTSGGGGSGGGGSGGGGSGGGGSGGGGSGGGGSEVQLLESGGGLVQPGGSLRLSCAASGFTFSSYWMSWVRQAPGKGLEWVSAISGSGGSTYYADSVKGRFTISRDNSKNTLYLQMNSLRAEDTAVYYCASSPLQWVDVWGQGTTVTVSSASTKGPSVFPLAPSSKSTSGGTAALGCLVKDYFPEPVTVSWNSGALTSGVHTFPAVLQSSGLYSLSSVVTVPSSSLGTQTYICNVNHKPSNTKVDKKVEPKSCDKTHTCPPCPAPEAAGGPSVFLFPPKPKDTLMISRTPEVTCVVVDVSHEDPEVKFNWYVDGVEVHNAKTKPREEQYNSTYRVVSVLTVLHQDWLNGKEYKCKVSNKALGAPIEKTISKAKGQPREPQVCTLPPSRDELTKNQVSLSCAVKGFYPSDIAVEWESNGQPENNYKTTPPVLDSDGSFFLVSKLTVDKSRWQQGNVFSCSVMHEALHNHYTQKSLSLSPGK

SEQ ID NO: 239 - protein, 688 aa, synthetic construct
  REGION 1..688: note = 65S-38B2 HC2-8 S354C/T366W LALAPG
ITCPPPMSVEHADIWVKSYSLYSRERYICNSGFKRKAGTSSLTECVLNKATNVAHWTTPSLKCIRDPALVHQRPAPPSGGGGSGGGGSGGGSGGGGSNWVNVISDLKKIEDLIQSMHIDATLYTESDVHPSCKVTAMKCFLLELQVISLESGDASIHDTVESLIILANNSLSSNGNVTESGCKECEELEEKNIKEFLQSFVHIVQMFINTSGGGGSGGGGSGGGGSGGGGSGGGGSGGGGSEVQLLESGGGLVQPGGSLRLSCAASGFTFSSYWMSWVRQAPGKGLEWVSAISGSGGSTYYADSVKGRFTISRDNSKNTLYLQMNSLRAEDTAVYYCASSPLQWVDVWGQGTTVTVSSASTKGPSVFPLAPSSKSTSGGTAALGCLVKDYFPEPVTVSWNSGALTSGVHTFPAVLQSSGLYSLSSVVTVPSSSLGTQTYICNVNHKPSNTKVDKKVEPKSCDKTHTCPPCPAPEAAGGPSVFLFPPKPKDTLMISRTPEVTCVVVDVSHEDPEVKFNWYVDGVEVHNAKTKPREEQYNSTYRVVSVLTVLHQDWLNGKEYKCKVSNKALGAPIEKTISKAKGQPREPQVYTLPPCRDELTKNQVSLWCLVKGFYPSDIAVEWESNGQPENNYKTTPPVLDSDGSFFLYSKLTVDKSRWQQGNVFSCSVMHEALHNHYTQKSLSLSPGK

SEQ ID NO: 240 - protein, 447 aa, synthetic construct
  REGION 1..447: note = 38B2 HC1-3B(CW-CSAV) S354C/T366W LALA
EVQLLESGGGLVQPGGSLRLSCAASGFTFSSYWMSWVRQAPGKGLEWVSAISGSGGSTYYADSVKGRFTISRDNSKNTLYLQMNSLRAEDTAVYYCASSPLQWVDVWGQGTTVTVSSASTKGPSVFPLAPSSKSTSGGTAALGCLVKDYFPEPVTVSWNSGALTSGVHTFPAVLQSSGLYSLSSVVTVPSSSLGTQTYICNVNHKPSNTKVDKKVEPKSCDKTHTCPPCPAPEAAGGPSVFLFPPKPKDTLMISRTPEVTCVVVDVSHEDPEVKFNWYVDGVEVHNAKTKPREEQYNSTYRVVSVLTVLHQDWLNGKEYKCKVSNKALPAPIEKTISKAKGQPREPQVYTLPPCRDELTKNQVSLWCLVKGFYPSDIAVEWESNGQPENNYKTTPPVLDSDGSFFLYSKLTVDKSRWQQGNVFSCSVMHEALHNHYTQKSLSLSPGK

SEQ ID NO: 241 - protein, 688 aa, synthetic construct
  REGION 1..688: note = 65S-38B2 HC2-3B(CW-CSAV) Y349C/T366S/L368A/Y407V LALA
ITCPPPMSVEHADIWVKSYSLYSRERYICNSGFKRKAGTSSLTECVLNKATNVAHWTTPSLKCIRDPALVHQRPAPPSGGSGGGGSGGGSGGGGSLQNWVNVISDLKKIEDLIQSMHIDATLYTESDVHPSCKVTAMKCFLLELQVISLESGDASIHDTVESLIILANNSLSSNGNVTESGCKECEELEEKNIKEFLQSFVHIVQMFINTSGGGGSGGGGSGGGGSGGGGSGGGGSGGGGSEVQLLESGGGLVQPGGSLRLSCAASGFTFSSYWMSWVRQAPGKGLEWVSAISGSGGSTYYADSVKGRFTISRDNSKNTLYLQMNSLRAEDTAVYYCASSPLQWVDVWGQGTTVTVSSASTKGPSVFPLAPSSKSTSGGTAALGCLVKDYFPEPVTVSWNSGALTSGVHTFPAVLQSSGLYSLSSVVTVPSSSLGTQTYICNVNHKPSNTKVDKKVEPKSCDKTHTCPPCPAPEAAGGPSVFLFPPKPKDTLMISRTPEVTCVVVDVSHEDPEVKFNWYVDGVEVHNAKTKPREEQYNSTYRVVSVLTVLHQDWLNGKEYKCKVSNKALPAPIEKTISKAKGQPREPQVCTLPPSRDELTKNQVSLSCAVKGFYPSDIAVEWESNGQPENNYKTTPPVLDSDGSFFLVSKLTVDKSRWQQGNVFSCSVMHEALHNHYTQKSLSLSPGK

SEQ ID NO: 242 - protein, 688 aa, synthetic construct
  REGION 1..688: note = 65S-38B2 HC2-7B(CW-CSAV) Y349C/T366S/L368A/Y407V LALA
ITCPPPMSVEHADIWVKSYSLYSRERYICNSGFKRKAGTSSLTECVLNKATNVAHWTTPSLKCIRDPALVHQRPAPPSGGGGSGGGGSGGGSGGGGSNWVNVISDLKKIEDLIQSMHIDATLYTESDVHPSCKVTAMKCFLLELQVISLESGDASIHDTVESLIILANNSLSSNGNVTESGCKECEELEEKNIKEFLQSFVHIVQMFINTSGGGGSGGGGSGGGGSGGGGSGGGGSGGGGSEVQLLESGGGLVQPGGSLRLSCAASGFTFSSYWMSWVRQAPGKGLEWVSAISGSGGSTYYADSVKGRFTISRDNSKNTLYLQMNSLRAEDTAVYYCASSPLQWVDVWGQGTTVTVSSASTKGPSVFPLAPSSKSTSGGTAALGCLVKDYFPEPVTVSWNSGALTSGVHTFPAVLQSSGLYSLSSVVTVPSSSLGTQTYICNVNHKPSNTKVDKKVEPKSCDKTHTCPPCPAPEAAGGPSVFLFPPKPKDTLMISRTPEVTCVVVDVSHEDPEVKFNWYVDGVEVHNAKTKPREEQYNSTYRVVSVLTVLHQDWLNGKEYKCKVSNKALPAPIEKTISKAKGQPREPQVCTLPPSRDELTKNQVSLSCAVKGFYPSDIAVEWESNGQPENNYKTTPPVLDSDGSFFLVSKLTVDKSRWQQGNVFSCSVMHEALHNHYTQKSLSLSPGK

SEQ ID NO: 243 - protein, 688 aa, synthetic construct
  REGION 1..688: note = 65D-38B2 HC2-3B(CW-CSAV) Y349C/T366S/L368A/Y407V LALA
ITCPPPMSVEHADIWVKSYSLYSRERYICNSGFKRKAGTSSLTECVLNKATNVAHWTTPSLKCIRDPALVHQRPAPPSGGSGGGGSGGGSGGGGSLQNWVNVISDLKKIEDLIQSMHIDATLYTESDVHPSCKVTAMKCFLLELQVISLESGDASIHDTVEDLIILANNSLSSNGNVTESGCKECEELEEKNIKEFLQSFVHIVQMFINTSGGGGSGGGGSGGGGSGGGGSGGGGSGGGGSEVQLLESGGGLVQPGGSLRLSCAASGFTFSSYWMSWVRQAPGKGLEWVSAISGSGGSTYYADSVKGRFTISRDNSKNTLYLQMNSLRAEDTAVYYCASSPLQWVDVWGQGTTVTVSSASTKGPSVFPLAPSSKSTSGGTAALGCLVKDYFPEPVTVSWNSGALTSGVHTFPAVLQSSGLYSLSSVVTVPSSSLGTQTYICNVNHKPSNTKVDKKVEPKSCDKTHTCPPCPAPEAAGGPSVFLFPPKPKDTLMISRTPEVTCVVVDVSHEDPEVKFNWYVDGVEVHNAKTKPREEQYNSTYRVVSVLTVLHQDWLNGKEYKCKVSNKALPAPIEKTISKAKGQPREPQVCTLPPSRDELTKNQVSLSCAVKGFYPSDIAVEWESNGQPENNYKTTPPVLDSDGSFFLVSKLTVDKSRWQQGNVFSCSVMHEALHNHYTQKSLSLSPGK

SEQ ID NO: 244 - protein, 20 aa, synthetic construct
  REGION 1..20: note = Exemplary linker
GGGGSGGGGSGGGGSGGGGS